European Patent Specification EP 3 433 280 B1, published April 19, 2023. Title: Protease-activated T cell bispecific molecules. Applicant: F.Hoffmann-La Roche Ltd. The sequence listing filed with the application follows.

SEQUENCE LISTING (170 sequences)

SEQ ID NO: 1 - protein, 215 aa, Chimeric
QAVVTQEPSLTVSPGGTVTLTCGSSTGAVTTSNYANWVQEKPGQAFRGLIGGTNKRAPGTPARFSGSLLGGKAALTLSGAQPEDEAEYYCALWYSNLWVFGGGTKLTVLGQPKAAPSVTLFPPSSEELQANKATLVCLISDFYPGAVTVAWKADSSPVKAGVETTTPSKQSNNKYAASSYLSLTPEQWKSHRSYSCQVTHEGSTVEKTVAPTECS

SEQ ID NO: 2 - protein, 971 aa, Chimeric
QIQLVQSGPELKKPGETVRISCKASGYTFTDYSIHWVKQAPGKCLKWMGWINTETGEPAYADDFKGRFAFSLETSASTAYLQINNLKNEDTATFFCAHPYDYDVLDYWGQGTSVTVSSGGGGSGGGGSGGGGSGGGGSDTVLTQSPASLGVSLGQRATISCRASKSVSTSNYSYIHWYQQKPGQPPKLLIKYVSYLESGVPARFSGSGSGTDFTLNIHPVEEEDAATYYCQHSREFPWTFGCGTKLEIKGGGGSGGGGSRQARVVNGGGGGSGGGGSGGGGSEVQLLESGGGLVQPGGSLRLSCAASGFTFSTYAMNWVRQAPGKGLEWVSRIRSKYNNYATYYADSVKGRFTISRDDSKNTLYLQMNSLRAEDTAVYYCVRHGNFGNSYVSWFAYWGQGTLVTVSSASTKGPSVFPLAPSSKSTSGGTAALGCLVKDYFPEPVTVSWNSGALTSGVHTFPAVLQSSGLYSLSSVVTVPSSSLGTQTYICNVNHKPSNTKVDKKVEPKSCDGGGGSGGGGSEVQLVESGGGLVKPGGSLRLSCAASGFTFSNAWMSWVRQAPGKGLEWVGRIKSKTDGGTTDYAAPVKGRFTISRDDSKNTLYLQMNSLKTEDTAVYYCTTPWEWSWYDYWGQGTLVTVSSASTKGPSVFPLAPSSKSTSGGTAALGCLVKDYFPEPVTVSWNSGALTSGVHTFPAVLQSSGLYSLSSVVTVPSSSLGTQTYICNVNHKPSNTKVDKKVEPKSCDKTHTCPPCPAPEAAGGPSVFLFPPKPKDTLMISRTPEVTCVVVDVSHEDPEVKFNWYVDGVEVHNAKTKPREEQYNSTYRVVSVLTVLHQDWLNGKEYKCKVSNKALGAPIEKTISKAKGQPREPQVYTLPPCRDELTKNQVSLWCLVKGFYPSDIAVEWESNGQPENNYKTTPPVLDSDGSFFLYSKLTVDKSRWQQGNVFSCSVMHEALHNHYTQKSLSLSPGK

SEQ ID NO: 3 - protein, 450 aa, Chimeric
EVQLVESGGGLVKPGGSLRLSCAASGFTFSNAWMSWVRQAPGKGLEWVGRIKSKTDGGTTDYAAPVKGRFTISRDDSKNTLYLQMNSLKTEDTAVYYCTTPWEWSWYDYWGQGTLVTVSSASTKGPSVFPLAPSSKSTSGGTAALGCLVKDYFPEPVTVSWNSGALTSGVHTFPAVLQSSGLYSLSSVVTVPSSSLGTQTYICNVNHKPSNTKVDKKVEPKSCDKTHTCPPCPAPEAAGGPSVFLFPPKPKDTLMISRTPEVTCVVVDVSHEDPEVKFNWYVDGVEVHNAKTKPREEQYNSTYRVVSVLTVLHQDWLNGKEYKCKVSNKALGAPIEKTISKAKGQPREPQVCTLPPSRDELTKNQVSLSCAVKGFYPSDIAVEWESNGQPENNYKTTPPVLDSDGSFFLVSKLTVDKSRWQQGNVFSCSVMHEALHNRFTQKSLSLSPGK

SEQ ID NO: 4 - protein, 971 aa, Chimeric
QVQLKESGPGLVAPSQSLSITCTVSGFSLTSYGVSWVRQPPGKCLEWLGIIWGDGSTNYHSALISRLSISKDNSKSQVFLKLNSLQTDDTATYYCAKGITTVVDDYYAMDYWGQGTSVTVSSGGGGSGGGGSGGGGSGGGGSDIQMTQSPASLSASVGETVTITCRASENIDSYLAWYQQKQGKSPQLLVYAATFLADDVPSRFSGSGSGTQYSLKINSLQSEDVARYYCQHYYSTPYTFGCGTKLEIKGGGGSGGGGSRQARVVNGGGGGSGGGGSGGGGSEVQLLESGGGLVQPGGSLRLSCAASGFTFSTYAMNWVRQAPGKGLEWVSRIRSKYNNYATYYADSVKGRFTISRDDSKNTLYLQMNSLRAEDTAVYYCVRHGNFGNSYVSWFAYWGQGTLVTVSSASTKGPSVFPLAPSSKSTSGGTAALGCLVKDYFPEPVTVSWNSGALTSGVHTFPAVLQSSGLYSLSSVVTVPSSSLGTQTYICNVNHKPSNTKVDKKVEPKSCDGGGGSGGGGSEVQLVESGGGLVKPGGSLRLSCAASGFTFSNAWMSWVRQAPGKGLEWVGRIKSKTDGGTTDYAAPVKGRFTISRDDSKNTLYLQMNSLKTEDTAVYYCTTPWEWSWYDYWGQGTLVTVSSASTKGPSVFPLAPSSKSTSGGTAALGCLVKDYFPEPVTVSWNSGALTSGVHTFPAVLQSSGLYSLSSVVTVPSSSLGTQTYICNVNHKPSNTKVDKKVEPKSCDKTHTCPPCPAPEAAGGPSVFLFPPKPKDTLMISRTPEVTCVVVDVSHEDPEVKFNWYVDGVEVHNAKTKPREEQYNSTYRVVSVLTVLHQDWLNGKEYKCKVSNKALGAPIEKTISKAKGQPREPQVYTLPPCRDELTKNQVSLWCLVKGFYPSDIAVEWESNGQPENNYKTTPPVLDSDGSFFLYSKLTVDKSRWQQGNVFSCSVMHEALHNHYTQKSLSLSPGK

SEQ ID NO: 5 - protein, 971 aa, Chimeric
QVQLKESGPGLVAPSQSLSITCTVSGFSLTSYGVSWVRQPPGKCLEWLGIIWGDGSTNYHSALISRLSISKDNSKSQVFLKLNSLQTDDTATYYCAKGITTVVDDYYAMDYWGQGTSVTVSSGGGGSGGGGSGGGGSGGGGSDIQMTQSPASLSASVGETVTITCRASENIDSYLAWYQQKQGKSPQLLVYAATFLADDVPSRFSGSGSGTQYSLKINSLQSEDVARYYCQHYYSTPYTFGCGTKLEIKGGGGSGGGGSGGGGSGGGGGGGSGGGGSGGGGSEVQLLESGGGLVQPGGSLRLSCAASGFTFSTYAMNWVRQAPGKGLEWVSRIRSKYNNYATYYADSVKGRFTISRDDSKNTLYLQMNSLRAEDTAVYYCVRHGNFGNSYVSWFAYWGQGTLVTVSSASTKGPSVFPLAPSSKSTSGGTAALGCLVKDYFPEPVTVSWNSGALTSGVHTFPAVLQSSGLYSLSSVVTVPSSSLGTQTYICNVNHKPSNTKVDKKVEPKSCDGGGGSGGGGSEVQLVESGGGLVKPGGSLRLSCAASGFTFSNAWMSWVRQAPGKGLEWVGRIKSKTDGGTTDYAAPVKGRFTISRDDSKNTLYLQMNSLKTEDTAVYYCTTPWEWSWYDYWGQGTLVTVSSASTKGPSVFPLAPSSKSTSGGTAALGCLVKDYFPEPVTVSWNSGALTSGVHTFPAVLQSSGLYSLSSVVTVPSSSLGTQTYICNVNHKPSNTKVDKKVEPKSCDKTHTCPPCPAPEAAGGPSVFLFPPKPKDTLMISRTPEVTCVVVDVSHEDPEVKFNWYVDGVEVHNAKTKPREEQYNSTYRVVSVLTVLHQDWLNGKEYKCKVSNKALGAPIEKTISKAKGQPREPQVYTLPPCRDELTKNQVSLWCLVKGFYPSDIAVEWESNGQPENNYKTTPPVLDSDGSFFLYSKLTVDKSRWQQGNVFSCSVMHEALHNHYTQKSLSLSPGK

SEQ ID NO: 6 - protein, 971 aa, Chimeric
QIQLVQSGPELKKPGETVRISCKASGYTFTDYSIHWVKQAPGKCLKWMGWINTETGEPAYADDFKGRFAFSLETSASTAYLQINNLKNEDTATFFCAHPYDYDVLDYWGQGTSVTVSSGGGGSGGGGSGGGGSGGGGSDTVLTQSPASLGVSLGQRATISCRASKSVSTSNYSYIHWYQQKPGQPPKLLIKYVSYLESGVPARFSGSGSGTDFTLNIHPVEEEDAATYYCQHSREFPWTFGCGTKLEIKGGGGSGGGGSGGGGSGGGGGGGSGGGGSGGGGSEVQLLESGGGLVQPGGSLRLSCAASGFTFSTYAMNWVRQAPGKGLEWVSRIRSKYNNYATYYADSVKGRFTISRDDSKNTLYLQMNSLRAEDTAVYYCVRHGNFGNSYVSWFAYWGQGTLVTVSSASTKGPSVFPLAPSSKSTSGGTAALGCLVKDYFPEPVTVSWNSGALTSGVHTFPAVLQSSGLYSLSSVVTVPSSSLGTQTYICNVNHKPSNTKVDKKVEPKSCDGGGGSGGGGSEVQLVESGGGLVKPGGSLRLSCAASGFTFSNAWMSWVRQAPGKGLEWVGRIKSKTDGGTTDYAAPVKGRFTISRDDSKNTLYLQMNSLKTEDTAVYYCTTPWEWSWYDYWGQGTLVTVSSASTKGPSVFPLAPSSKSTSGGTAALGCLVKDYFPEPVTVSWNSGALTSGVHTFPAVLQSSGLYSLSSVVTVPSSSLGTQTYICNVNHKPSNTKVDKKVEPKSCDKTHTCPPCPAPEAAGGPSVFLFPPKPKDTLMISRTPEVTCVVVDVSHEDPEVKFNWYVDGVEVHNAKTKPREEQYNSTYRVVSVLTVLHQDWLNGKEYKCKVSNKALGAPIEKTISKAKGQPREPQVYTLPPCRDELTKNQVSLWCLVKGFYPSDIAVEWESNGQPENNYKTTPPVLDSDGSFFLYSKLTVDKSRWQQGNVFSCSVMHEALHNHYTQKSLSLSPGK

SEQ ID NO: 7 - protein, 33 aa, Chimeric
GGGGSGGGGSRQARVVNGGGGGSGGGGSGGGGS

SEQ ID NO: 8 - protein, 28 aa, Chimeric
GGGGSVHMPLGFLGPGRSRGSFPGGGGS

SEQ ID NO: 9 - protein, 41 aa, Chimeric
GGGGSGGGGSRQARVVNGGGGGSVPLSLYSGGGGGSGGGGS

SEQ ID NO: 10 - protein, 36 aa, Chimeric
GGGGSGGGGSRQARVVNGVPLSLYSGGGGGSGGGGS

SEQ ID NO: 11 - protein, 5 aa, Chimeric
TYAMN

SEQ ID NO: 12 - protein, 19 aa, Chimeric
RIRSKYNNYATYYADSVKG

SEQ ID NO: 13 - protein, 14 aa, Chimeric
HGNFGNSYVSWFAY

SEQ ID NO: 14 - protein, 5 aa, Chimeric
NAWMS

SEQ ID NO: 15 - protein, 19 aa, Chimeric
RIKSKTDGGTTDYAAPVKG

SEQ ID NO: 16 - protein, 9 aa, Chimeric
PWEWSWYDY

SEQ ID NO: 17 - protein, 14 aa, Chimeric
GSSTGAVTTSNYAN

SEQ ID NO: 18 - protein, 7 aa, Chimeric
GTNKRAP

SEQ ID NO: 19 - protein, 9 aa, Chimeric
ALWYSNLWV

SEQ ID NO: 20 - protein, 5 aa, Chimeric
DYSIH

SEQ ID NO: 21 - protein, 17 aa, Chimeric
WINTETGEPAYADDFKG

SEQ ID NO: 22 - protein, 9 aa, Chimeric
PYDYDVLDY

SEQ ID NO: 23 - protein, 15 aa, Chimeric
RASKSVSTSNYSYIH

SEQ ID NO: 24 - protein, 7 aa, Chimeric
YVSYLES

SEQ ID NO: 25 - protein, 9 aa, Chimeric
QHSREFPWT

SEQ ID NO: 26 - protein, 5 aa, Chimeric
SYGVS

SEQ ID NO: 27 - protein, 16 aa, Chimeric
IIWGDGSTNYHSALIS

SEQ ID NO: 28 - protein, 14 aa, Chimeric
GITTVVDDYYAMDY

SEQ ID NO: 29 - protein, 11 aa, Chimeric
RASENIDSYLA

SEQ ID NO: 30 - protein, 7 aa, Chimeric
AATFLAD

SEQ ID NO: 31 - protein, 9 aa, Chimeric
QHYYSTPYT

SEQ ID NO: 32 - protein, 450 aa, Chimeric
QVQLVQSGAEVKKPGSSVKVSCKASGFTFTDYKIHWVRQAPGQGLEWMGYFNPNSGYSTYAQKFQGRVTITADKSTSTAYMELSSLRSEDTAVYYCARLSPGGYYVMDAWGQGTTVTVSSASTKGPSVFPLAPSSKSTSGGTAALGCLVKDYFPEPVTVSWNSGALTSGVHTFPAVLQSSGLYSLSSVVTVPSSSLGTQTYICNVNHKPSNTKVDKKVEPKSCDKTHTCPPCPAPELLGGPSVFLFPPKPKDTLMISRTPEVTCVVVDVSHEDPEVKFNWYVDGVEVHNAKTKPREEQYNSTYRVVSVLTVLHQDWLNGKEYKCKVSNKALPAPIEKTISKAKGQPREPQVYTLPPSRDELTKNQVSLTCLVKGFYPSDIAVEWESNGQPENNYKTTPPVLDSDGSFFLYSKLTVDKSRWQQGNVFSCSVMHEALHNHYTQKSLSLSPGK

SEQ ID NO: 33 - protein, 213 aa, Chimeric
DIQMTQSPSSLSASVGDRVTITCRASQGINNYLNWYQQKPGKAPKRLIYNTNNLQTGVPSRFSGSGSGTEFTLTISSLQPEDFATYYCLQHNSFPTFGQGTKLEIKRTVAAPSVFIFPPSDEQLKSGTASVVCLLNNFYPREAKVQWKVDNALQSGNSQESVTEQDSKDSTYSLSSTLTLSKADYEKHKVYACEVTHQGLSSPVTKSFNRGEC

SEQ ID NO: 34 - protein, 492 aa, Chimeric
EVQLEQSGPVLVKPGTSVKMSCKASGYTFTDYYINWIIQSHGKCLEWIGVINPDSGGTDYNQNFKGKATLTVDKSSTTAYMELTSLTSEDSAVYYCARRDSYGFDYWGQGTTLTVSSGGGGSGGGGSGGGGSGGGGSDIVLTQTPKFLLVPAGDRITMTCKASLSVTNDVAWYQQKPGQSPKLLLYYASNRNAGVPDRFTGSGYGTDFTFTITTLQAEDLAVYFCQQDYTSPPTFGCGTKLEIRGGGGSGGGGSGPLGLWSQGGGGSGGGGSGGGGSGGDIQMTQSPSSLSASVGDRVTITCRASQGINNYLNWYQQKPGKAPKRLIYNTNNLQTGVPSRFSGSGSGTEFTLTISSLQPEDFATYYCLQHNSFPTFGQGTKLEIKRTVAAPSVFIFPPSDEQLKSGTASVVCLLNNFYPREAKVQWKVDNALQSGNSQESVTEQDSKDSTYSLSSTLTLSKADYEKHKVYACEVTHQGLSSPVTKSFNRGEC

SEQ ID NO: 35 - protein, 35 aa, Chimeric
GGGGSGGGGSGPLGLWSQGGGGSGGGGSGGGGSGG

SEQ ID NO: 36 - protein, 8 aa, Chimeric
RQARVVNG

SEQ ID NO: 37 - protein, 18 aa, Chimeric
VHMPLGFLGPGRSRGSFP

SEQ ID NO: 38 - protein, 21 aa, Chimeric
  X (9)..(13): X is an amino acid
  X (9)..(13): X or Xaa is an amino acid
RQARVVNGXXXXXVPLSLYSG

SEQ ID NO: 39 - protein, 16 aa, Chimeric
RQARVVNGVPLSLYSG

SEQ ID NO: 40 - protein, 7 aa, Chimeric
PLGLWSQ

SEQ ID NO: 41 - protein, 249 aa, Chimeric
QIQLVQSGPELKKPGETVRISCKASGYTFTDYSIHWVKQAPGKCLKWMGWINTETGEPAYADDFKGRFAFSLETSASTAYLQINNLKNEDTATFFCAHPYDYDVLDYWGQGTSVTVSSGGGGSGGGGSGGGGSGGGGSDTVLTQSPASLGVSLGQRATISCRASKSVSTSNYSYIHWYQQKPGQPPKLLIKYVSYLESGVPARFSGSGSGTDFTLNIHPVEEEDAATYYCQHSREFPWTFGCGTKLEIK

SEQ ID NO: 42 - protein, 249 aa, Chimeric
QVQLKESGPGLVAPSQSLSITCTVSGFSLTSYGVSWVRQPPGKCLEWLGIIWGDGSTNYHSALISRLSISKDNSKSQVFLKLNSLQTDDTATYYCAKGITTVVDDYYAMDYWGQGTSVTVSSGGGGSGGGGSGGGGSGGGGSDIQMTQSPASLSASVGETVTITCRASENIDSYLAWYQQKQGKSPQLLVYAATFLADDVPSRFSGSGSGTQYSLKINSLQSEDVARYYCQHYYSTPYTFGCGTKLEIK

SEQ ID NO: 43 - protein, 125 aa, Chimeric
EVQLLESGGGLVQPGGSLRLSCAASGFTFSTYAMNWVRQAPGKGLEWVSRIRSKYNNYATYYADSVKGRFTISRDDSKNTLYLQMNSLRAEDTAVYYCVRHGNFGNSYVSWFAYWGQGTLVTVSS

SEQ ID NO: 44 - protein, 5 aa, Chimeric
TYAMN

SEQ ID NO: 45 - protein, 19 aa, Chimeric
RIRSKYNNYATYYADSVKG

SEQ ID NO: 46 - protein, 14 aa, Chimeric
HGNFGNSYVSWFAY

SEQ ID NO: 47 - protein, 120 aa, Chimeric
EVQLVESGGGLVKPGGSLRLSCAASGFTFSNAWMSWVRQAPGKGLEWVGRIKSKTDGGTTDYAAPVKGRFTISRDDSKNTLYLQMNSLKTEDTAVYYCTTPWEWSWYDYWGQGTLVTVSS

SEQ ID NO: 48 - protein, 5 aa, Chimeric
DYYIN

SEQ ID NO: 49 - protein, 17 aa, Chimeric
VINPDSGGTDYNQNFKG

SEQ ID NO: 50 - protein, 8 aa, Chimeric
RDSYGFDY

SEQ ID NO: 51 - protein, 11 aa, Chimeric
KASLSVTNDVA

SEQ ID NO: 52 - protein, 7 aa, Chimeric
YASNRNA

SEQ ID NO: 53 - protein, 9 aa, Chimeric
QQDYTSPPT

SEQ ID NO: 54 - protein, 207 aa, Homo sapiens
MQSGTHWRVLGLCLLSVGVWGQDGNEEMGGITQTPYKVSISGTTVILTCPQYPGSEILWQHNDKNIGGDEDDKNIGSDEDHLSLKEFSELEQSGYYVCYPRGSKPEDANFYLYLRARVCENCMEMDVMSVATIVIVDICITGGLLLLVYYWSKNRKAKAKPVTRGAGAGGRQRGQNKERPPPVPNPDYEPIRKGQRDLYSGLNQRRI

SEQ ID NO: 55 - protein, 109 aa, Chimeric
QAVVTQEPSLTVSPGGTVTLTCGSSTGAVTTSNYANWVQEKPGQAFRGLIGGTNKRAPGTPARFSGSLLGGKAALTLSGAQPEDEAEYYCALWYSNLWVFGGGTKLTVL

SEQ ID NO: 56 - protein, 5 aa, Chimeric
DYKIH

SEQ ID NO: 57 - protein, 17 aa, Chimeric
YFNPNSGYSTYAQKFQG

SEQ ID NO: 58 - protein, 11 aa, Chimeric
LSPGGYYVMDA

SEQ ID NO: 59 - protein, 11 aa, Chimeric
RASQGINNYLN

SEQ ID NO: 60 - protein, 7 aa, Chimeric
NTNNLQT

SEQ ID NO: 61 - protein, 8 aa, Chimeric
LQHNSFPT

SEQ ID NO: 62 - DNA, 648 bp, Chimeric
caggccgtcgtgacccaggaacccagcctgacagtgtctcctggcggcaccgtgaccctgacatgtggcagttctacaggcgccgtgaccaccagcaactacgccaactgggtgcaggaaaagcccggccaggccttcagaggactgatcggcggcaccaacaagagagcccctggcacccctgccagattcagcggatctctgctgggaggaaaggccgccctgacactgtctggcgcccagccagaagatgaggccgagtactactgcgccctgtggtacagcaacctgtgggtgttcggcggaggcaccaagctgacagtcctaggtcaacccaaggctgcccccagcgtgaccctgttcccccccagcagcgaggaactgcaggccaacaaggccaccctggtctgcctgatcagcgacttctacccaggcgccgtgaccgtggcctggaaggccgacagcagccccgtgaaggccggcgtggagaccaccacccccagcaagcagagcaacaacaagtacgccgccagcagctacctgagcctgacccccgagcagtggaagagccacaggtcctacagctgccaggtgacccacgagggcagcaccgtggagaaaaccgtggcccccaccgagtgcagctga

SEQ ID NO: 63 - DNA, 2916 bp, Chimeric
cagatccagctggtgcagagcggccctgagctgaagaaacccggcgagacagtgcggatcagctgcaaggccagcggctacaccttcaccgactacagcatccactgggtcaagcaggcccctggcaagtgcctgaagtggatgggctggatcaacaccgagacaggcgagcccgcctacgccgacgatttcaagggcagattcgccttcagcctggaaaccagcgccagcaccgcctacctgcagatcaacaacctgaagaacgaggacaccgccacctttttctgcgcccacccctacgactacgacgtgctggattattggggccagggcaccagcgtgaccgtgtctagcggaggcggaggatctggcggcggaggaagtggcggagggggatctgggggaggcggatctgataccgtgctgacacagagccctgccagcctgggagtgtccctgggacagagagccaccatcagctgtcgggccagcaagagcgtgtccaccagcaactacagctatatccactggtatcagcagaagcccggccagccccccaagctgctgatcaaatacgtgtcctacctggaaagcggcgtgcccgccagattttctggctctggcagcggcaccgacttcaccctgaacatccaccccgtggaagaggaagatgccgccacctactactgccagcacagcagagagttcccttggaccttcggctgcggcaccaagctggaaatcaaaggcgggggaggctccggaggcggcggaagtagacaggccagagtcgtgaacgggggaggggggggaagtgggggcggaggcagtggggggggaggatccgaggtgcagctgctggaatctggcggcggactggtgcagcctggcggatctctgagactgagctgtgccgccagcggcttcaccttcagcacctacgccatgaactgggtgcgccaggcccctggcaaaggcctggaatgggtgtcccggatcagaagcaagtacaacaactacgccacctactacgccgacagcgtgaagggccggttcaccatcagccgggacgacagcaagaacaccctgtacctgcagatgaacagcctgcgggccgaggacaccgccgtgtactattgtgtgcggcacggcaacttcggcaacagctatgtgtcttggtttgcctactggggccagggcaccctcgtgaccgtgtcaagcgctagcacaaagggccctagcgtgttccctctggcccccagcagcaagagcacaagcggcggaacagccgccctgggctgcctcgtgaaggactacttccccgagcccgtgacagtgtcttggaacagcggagccctgacaagcggcgtgcacaccttccctgccgtgctgcagagcagcggcctgtactccctgagcagcgtggtcaccgtgcctagcagcagcctgggcacccagacctacatctgcaacgtgaaccacaagcccagcaacaccaaagtggacaagaaggtggagcccaagagctgtgatggcggaggagggtccggaggcggaggatccgaggtgcaattggttgaatctggtggtggtctggtaaaaccgggcggttccctgcgtctgagctgcgcggcttccggattcaccttctccaacgcgtggatgagctgggttcgccaggccccgggcaaaggcctcgagtgggttggtcgtatcaagtctaaaactgacggtggcaccacggattacgcggctccagttaaaggtcgttttaccatttcccgcgacgatagcaaaaacactctgtatctgcagatgaactctctgaaaactgaagacaccgcagtctactactgtactaccccgtgggaatggtcttggtacgattattggggccagggcacgctggttacggtgtctagcgctagtaccaagggccccagcgtgttccccctggcacccagcagcaagagcacatctggcggaacagccgctctgggctgtctggtgaaagactacttccccgagcccgtgaccgtgtcttggaactctggcgccctgaccagcggcgtgcacacctttccagccgtgctgcagagcagcggcctgtactccctgtcctccgtggtcaccgtgccctctagctccctgggaacacagacatatatctgtaatgtcaatcacaagccttccaacaccaaagtcgataagaaagtcgagcccaagagctgcgacaaaactcacacatgcccaccgtgcccagcacctgaagctgcagggggaccgtcagtcttcctcttccccccaaaacccaaggacaccctcatgatctcccggacccctgaggtcacatgcgtggtggtggacgtgagccacgaagaccctgaggtcaagttcaactggtacgtggacggcgtggaggtgcataatgccaagacaaagccgcgggaggagcagtacaacagcacgtaccgtgtggtcagcgtcctcaccgtcctgcaccaggactggctgaatggcaaggagtacaagtgcaaggtctccaacaaagccctcggcgcccccatcgagaaaaccatctccaaagccaaagggcagccccgagaaccacaggtgtacaccctgcccccatgccgggatgagctgaccaagaaccaggtcagcctgtggtgcctggtcaaaggcttctatcccagcgacatcgccgtggagtgggagagcaatgggcagccggagaacaactacaagaccacgcctcccgtgctggactccgacggctccttcttcctctacagcaagctcaccgtggacaagagcaggtggcagcaggggaacgtcttctcatgctccgtgatgcatgaggctctgcacaaccactacacgcagaagagcctctccctgtctccgggtaaatga

SEQ ID NO: 64 - DNA, 1353 bp, Chimeric
gaggtgcaattggttgaatctggtggtggtctggtaaaaccgggcggttccctgcgtctgagctgcgcggcttccggattcaccttctccaacgcgtggatgagctgggttcgccaggccccgggcaaaggcctcgagtgggttggtcgtatcaagtctaaaactgacggtggcaccacggattacgcggctccagttaaaggtcgttttaccatttcccgcgacgatagcaaaaacactctgtatctgcagatgaactctctgaaaactgaagacaccgcagtctactactgtactaccccgtgggaatggtcttggtacgattattggggccagggcacgctggttacggtgtcttccgctagcaccaagggcccctccgtgttccccctggcccccagcagcaagagcaccagcggcggcacagccgctctgggctgcctggtcaaggactacttccccgagcccgtgaccgtgtcctggaacagcggagccctgacctccggcgtgcacaccttccccgccgtgctgcagagttctggcctgtatagcctgagcagcgtggtcaccgtgccttctagcagcctgggcacccagacctacatctgcaacgtgaaccacaagcccagcaacaccaaggtggacaagaaggtggagcccaagagctgcgacaaaactcacacatgcccaccgtgcccagcacctgaagctgcagggggaccgtcagtcttcctcttccccccaaaacccaaggacaccctcatgatctcccggacccctgaggtcacatgcgtggtggtggacgtgagccacgaagaccctgaggtcaagttcaactggtacgtggacggcgtggaggtgcataatgccaagacaaagccgcgggaggagcagtacaacagcacgtaccgtgtggtcagcgtcctcaccgtcctgcaccaggactggctgaatggcaaggagtacaagtgcaaggtctccaacaaagccctcggcgcccccatcgagaaaaccatctccaaagccaaagggcagccccgagaaccacaggtgtgcaccctgcccccatcccgggatgagctgaccaagaaccaggtcagcctctcgtgcgcagtcaaaggcttctatcccagcgacatcgccgtggagtgggagagcaatgggcagccggagaacaactacaagaccacgcctcccgtgctggactccgacggctccttcttcctcgtgagcaagctcaccgtggacaagagcaggtggcagcaggggaacgtcttctcatgctccgtgatgcatgaggctctgcacaaccgcttcacgcagaagagcctctccctgtctccgggtaaatga

SEQ ID NO: 65 - DNA, 2916 bp, Chimeric
caagtgcagctgaaagagtccggccctggactggtggcccctagccagagcctgagcatcacctgtaccgtgtccggcttcagcctgaccagctacggcgtgtcatgggtgcgccagcctccaggcaagtgtctggaatggctgggcatcatctggggcgacggcagcaccaattaccacagcgccctgatcagcagactgagcatctccaaggacaacagcaagagccaggtgttcctgaagctgaacagcctgcagaccgacgacaccgccacctactactgcgccaagggcatcaccaccgtggtggacgactactacgctatggactactggggccagggcaccagcgtgacagtgtctagcggaggcggaggatctggcggcggaggaagtggcggagggggatctgggggaggcggaagcgatatccagatgacccagagccctgccagcctgtctgcctctgtgggcgagacagtgaccatcacatgccgggccagcgagaacatcgacagctacctggcctggtatcagcagaagcagggcaagagcccccagctgctggtgtacgccgccacctttctggccgacgatgtgcccagcagattcagcggcagcggaagcggcacacagtacagcctgaagatcaactccctgcagagcgaggacgtggcccggtactactgccagcactactacagcaccccctacaccttcggctgcggcaccaagctggaaatcaaaggcgggggaggctccggaggcggcggaagtagacaggccagagtcgtgaacgggggaggggggggaagtgggggcggaggcagtgggggcggaggatccgaggtgcagctgctggaatctggcggcggactggtgcagcctggcggatctctgagactgagctgtgccgccagcggcttcaccttcagcacctacgccatgaactgggtgcgccaggcccctggcaaaggcctggaatgggtgtcccggatcagaagcaagtacaacaactacgccacctactacgccgacagcgtgaagggccggttcaccatcagccgggacgacagcaagaacaccctgtacctgcagatgaacagcctgcgggccgaggacaccgccgtgtactattgtgtgcggcacggcaacttcggcaacagctatgtgtcttggtttgcctactggggccagggcaccctcgtgaccgtgtcaagcgctagcacaaagggccctagcgtgttccctctggcccccagcagcaagagcacaagcggcggaacagccgccctgggctgcctcgtgaaggactacttccccgagcccgtgacagtgtcttggaacagcggagccctgacaagcggcgtgcacaccttccctgccgtgctgcagagcagcggcctgtactccctgagcagcgtggtcaccgtgcctagcagcagcctgggcacccagacctacatctgcaacgtgaaccacaagcccagcaacaccaaagtggacaagaaggtggagcccaagagctgtgatggcggaggagggtccgggggcggaggatccgaggtgcaattggttgaatctggtggtggtctggtaaaaccgggcggttccctgcgtctgagctgcgcggcttccgggttcaccttctccaacgcgtggatgagctgggttcgccaggccccgggcaaaggcctcgagtgggttggtcgtatcaagtctaaaactgacggtggcaccacggattacgcggctccagttaaaggtcgttttaccatttcccgcgacgatagcaaaaacactctgtatctgcagatgaactctctgaaaactgaagacaccgcagtctactactgtactaccccgtgggaatggtcttggtacgattattggggccagggcacgctggttacggtgtctagcgctagtaccaagggccccagcgtgttccccctggcacccagcagcaagagcacatctggcggaacagccgctctgggctgtctggtgaaagactacttccccgagcccgtgaccgtgtcttggaactctggcgccctgaccagcggcgtgcacacctttccagccgtgctgcagagcagcggcctgtactccctgtcctccgtggtcaccgtgccctctagctccctgggaacacagacatatatctgtaatgtcaatcacaagccttccaacaccaaagtcgataagaaagtcgagcccaagagctgcgacaaaactcacacatgcccaccgtgcccagcacctgaagctgcagggggaccgtcagtcttcctcttccccccaaaacccaaggacaccctcatgatctcccggacccctgaggtcacatgcgtggtggtggacgtgagccacgaagaccctgaggtcaagttcaactggtacgtggacggcgtggaggtgcataatgccaagacaaagccgcgggaggagcagtacaacagcacgtaccgtgtggtcagcgtcctcaccgtcctgcaccaggactggctgaatggcaaggagtacaagtgcaaggtctccaacaaagccctcggcgcccccatcgagaaaaccatctccaaagccaaagggcagccccgagaaccacaggtgtacaccctgcccccatgccgggatgagctgaccaagaaccaggtcagcctgtggtgcctggtcaaaggcttctatcccagcgacatcgccgtggagtgggagagcaatgggcagccggagaacaactacaagaccacgcctcccgtgctggactccgacggctccttcttcctctacagcaagctcaccgtggacaagagcaggtggcagcaggggaacgtcttctcatgctccgtgatgcatgaggctctgcacaaccactacacgcagaagagcctctccctgtctccgggtaaatga

SEQ ID NO: 66 - DNA, 2916 bp, Chimeric
caagtgcagctgaaagagtccggccctggactggtggcccctagccagagcctgagcatcacctgtaccgtgtccggcttcagcctgaccagctacggcgtgtcatgggtgcgccagcctccaggcaagtgtctggaatggctgggcatcatctggggcgacggcagcaccaattaccacagcgccctgatcagcagactgagcatctccaaggacaacagcaagagccaggtgttcctgaagctgaacagcctgcagaccgacgacaccgccacctactactgcgccaagggcatcaccaccgtggtggacgactactacgctatggactactggggccagggcaccagcgtgacagtgtctagcggaggcggaggatctggcggcggaggaagtggcggagggggatctgggggaggcggaagcgatatccagatgacccagagccctgccagcctgtctgcctctgtgggcgagacagtgaccatcacatgccgggccagcgagaacatcgacagctacctggcctggtatcagcagaagcagggcaagagcccccagctgctggtgtacgccgccacctttctggccgacgatgtgcccagcagattcagcggcagcggaagcggcacacagtacagcctgaagatcaactccctgcagagcgaggacgtggcccggtactactgccagcactactacagcaccccctacaccttcggctgcggcaccaagctggaaatcaaaggcgggggaggctccggaggcggcggaagtggaggcggcggaagtggcggaggcggaggggggggaagtgggggcggaggcagtggggggggaggatccgaggtgcagctgctggaatctggcggcggactggtgcagcctggcggatctctgagactgagctgtgccgccagcggcttcaccttcagcacctacgccatgaactgggtgcgccaggcccctggcaaaggcctggaatgggtgtcccggatcagaagcaagtacaacaactacgccacctactacgccgacagcgtgaagggccggttcaccatcagccgggacgacagcaagaacaccctgtacctgcagatgaacagcctgcgggccgaggacaccgccgtgtactattgtgtgcggcacggcaacttcggcaacagctatgtgtcttggtttgcctactggggccagggcaccctcgtgaccgtgtcaagcgctagcacaaagggccctagcgtgttccctctggcccccagcagcaagagcacaagcggcggaacagccgccctgggctgcctcgtgaaggactacttccccgagcccgtgacagtgtcttggaacagcggagccctgacaagcggcgtgcacaccttccctgccgtgctgcagagcagcggcctgtactccctgagcagcgtggtcaccgtgcctagcagcagcctgggcacccagacctacatctgcaacgtgaaccacaagcccagcaacaccaaagtggacaagaaggtggagcccaagagctgtgatggcggaggagggtccggaggcggaggctccgaggtgcaattggttgaatctggtggtggtctggtaaaaccgggcggttccctgcgtctgagctgcgcggcttccggattcaccttctccaacgcgtggatgagctgggttcgccaggccccgggcaaaggcctcgagtgggttggtcgtatcaagtctaaaactgacggtggcaccacggattacgcggctccagttaaaggtcgttttaccatttcccgcgacgatagcaaaaacactctgtatctgcagatgaactctctgaaaactgaagacaccgcagtctactactgtactaccccgtgggaatggtcttggtacgattattggggccagggcacgctggttacggtgtctagcgctagtaccaagggccccagcgtgttccccctggcacccagcagcaagagcacatctggcggaacagccgctctgggctgtctggtgaaagactacttccccgagcccgtgaccgtgtcttggaactctggcgccctgaccagcggcgtgcacacctttccagccgtgctgcagagcagcggcctgtactccctgtcctccgtggtcaccgtgccctctagctccctgggaacacagacatatatctgtaatgtcaatcacaagccttccaacaccaaagtcgataagaaagtcgagcccaagagctgcgacaaaactcacacatgcccaccgtgcccagcacctgaagctgcagggggaccgtcagtcttcctcttccccccaaaacccaaggacaccctcatgatctcccggacccctgaggtcacatgcgtggtggtggacgtgagccacgaagaccctgaggtcaagttcaactggtacgtggacggcgtggaggtgcataatgccaagacaaagccgcgggaggagcagtacaacagcacgtaccgtgtggtcagcgtcctcaccgtcctgcaccaggactggctgaatggcaaggagtacaagtgcaaggtctccaacaaagccctcggcgcccccatcgagaaaaccatctccaaagccaaagggcagccccgagaaccacaggtgtacaccctgcccccatgccgggatgagctgaccaagaaccaggtcagcctgtggtgcctggtcaaaggcttctatcccagcgacatcgccgtggagtgggagagcaatgggcagccggagaacaactacaagaccacgcctcccgtgctggactccgacggctccttcttcctctacagcaagctcaccgtggacaagagcaggtggcagcaggggaacgtcttctcatgctccgtgatgcatgaggctctgcacaaccactacacgcagaagagcctctccctgtctccgggtaaatga

SEQ ID NO: 67 - DNA, 2916 bp, Chimeric
cagatccagctggtgcagagcggccctgagctgaagaaacccggcgagacagtgcggatcagctgcaaggccagcggctacaccttcaccgactacagcatccactgggtcaagcaggcccctggcaagtgcctgaagtggatgggctggatcaacaccgagacaggcgagcccgcctacgccgacgatttcaagggcagattcgccttcagcctggaaaccagcgccagcaccgcctacctgcagatcaacaacctgaagaacgaggacaccgccacctttttctgcgcccacccctacgactacgacgtgctggattattggggccagggcaccagcgtgaccgtgtctagcggaggcggaggatctggcggcggaggaagtggcggagggggatctgggggaggcggatctgataccgtgctgacacagagccctgccagcctgggagtgtccctgggacagagagccaccatcagctgtcgggccagcaagagcgtgtccaccagcaactacagctatatccactggtatcagcagaagcccggccagccccccaagctgctgatcaaatacgtgtcctacctggaaagcggcgtgcccgccagattttctggctctggcagcggcaccgacttcaccctgaacatccaccccgtggaagaggaagatgccgccacctactactgccagcacagcagagagttcccttggaccttcggctgcggcaccaagctggaaatcaaaggcgggggaggctccggaggcggcggaagtggaggcggcggaagtggcggaggcggaggggggggaagtgggggcggaggcagtggggggggaggatccgaggtgcagctgctggaatctggcggcggactggtgcagcctggcggatctctgagactgagctgtgccgccagcggcttcaccttcagcacctacgccatgaactgggtgcgccaggcccctggcaaaggcctggaatgggtgtcccggatcagaagcaagtacaacaactacgccacctactacgccgacagcgtgaagggccggttcaccatcagccgggacgacagcaagaacaccctgtacctgcagatgaacagcctgcgggccgaggacaccgccgtgtactattgtgtgcggcacggcaacttcggcaacagctatgtgtcttggtttgcctactggggccagggcaccctcgtgaccgtgtcaagcgctagcacaaagggccctagcgtgttccctctggcccccagcagcaagagcacaagcggcggaacagccgccctgggctgcctcgtgaaggactacttccccgagcccgtgacagtgtcttggaacagcggagccctgacaagcggcgtgcacaccttccctgccgtgctgcagagcagcggcctgtactccctgagcagcgtggtcaccgtgcctagcagcagcctgggcacccagacctacatctgcaacgtgaaccacaagcccagcaacaccaaagtggacaagaaggtggagcccaagagctgtgatggcggaggagggtccggaggcggaggctccgaggtgcaattggttgaatctggtggtggtctggtaaaaccgggcggttccctgcgtctgagctgcgcggcttccggattcaccttctccaacgcgtggatgagctgggttcgccaggccccgggcaaaggcctcgagtgggttggtcgtatcaagtctaaaactgacggtggcaccacggattacgcggctccagttaaaggtcgttttaccatttcccgcgacgatagcaaaaacactctgtatctgcagatgaactctctgaaaactgaagacaccgcagtctactactgtactaccccgtgggaatggtcttggtacgattattggggccagggcacgctggttacggtgtctagcgctagtaccaagggccccagcgtgttccccctggcacccagcagcaagagcacatctggcggaacagccgctctgggctgtctggtgaaagactacttccccgagcccgtgaccgtgtcttggaactctggcgccctgaccagcggcgtgcacacctttccagccgtgctgcagagcagcggcctgtactccctgtcctccgtggtcaccgtgccctctagctccctgggaacacagacatatatctgtaatgtcaatcacaagccttccaacaccaaagtcgataagaaagtcgagcccaagagctgcgacaaaactcacacatgcccaccgtgcccagcacctgaagctgcagggggaccgtcagtcttcctcttccccccaaaacccaaggacaccctcatgatctcccggacccctgaggtcacatgcgtggtggtggacgtgagccacgaagaccctgaggtcaagttcaactggtacgtggacggcgtggaggtgcataatgccaagacaaagccgcgggaggagcagtacaacagcacgtaccgtgtggtcagcgtcctcaccgtcctgcaccaggactggctgaatggcaaggagtacaagtgcaaggtctccaacaaagccctcggcgcccccatcgagaaaaccatctccaaagccaaagggcagccccgagaaccacaggtgtacaccctgcccccatgccgggatgagctgaccaagaaccaggtcagcctgtggtgcctggtcaaaggcttctatcccagcgacatcgccgtggagtgggagagcaatgggcagccggagaacaactacaagaccacgcctcccgtgctggactccgacggctccttcttcctctacagcaagctcaccgtggacaagagcaggtggcagcaggggaacgtcttctcatgctccgtgatgcatgaggctctgcacaaccactacacgcagaagagcctctccctgtctccgggtaaatga

SEQ ID NO: 68 - DNA, 99 bp, Chimeric
ggcgggggaggctccggaggcggcggaagtagacaggccagagtcgtgaacgggggaggggggggaagtgggggcggaggcagtgggggcggaggatcc

SEQ ID NO: 69 - DNA, 1350 bp, Chimeric
caggtgcagctggtccagagcggcgccgaggtgaagaaacccgggtcctctgtcaaggtgtcatgcaaggctagcggattcacctttacagactacaaaatccactgggttaggcaggcacctggccaaggactcgaatggatggggtatttcaacccaaattccggctactctacctatgcccagaagtttcagggaagagtgactattacagctgataagagtaccagcactgcatacatggagctgtcctctcttcgctcagaggacaccgccgtctactattgtgctcggctgagccccggtggctactatgtgatggatgcatgggggcagggaacaaccgtaacagtgtcctctgcgtcgactaagggcccttcagtttttccactcgcccccagtagcaagtccacatctgggggtaccgctgccctgggctgccttgtgaaagactatttccctgaaccagtcactgtgtcatggaatagcggagccctgacctccggtgtacacacattccccgctgtgttgcagtctagtggcctgtacagcctctcctctgttgtgaccgtcccttcaagctccctggggacacagacctatatctgtaacgtgaatcataagccatctaacactaaagtagataaaaaagtggagcccaagagttgcgacaaaacacacacctgtcccccttgcccagcccccgagcttctgggaggccctagcgtctttctcttcccacccaagcctaaggatactctgatgatatccaggaccccagaagttacatgcgtggtcgtggacgtctcacacgaggaccccgaagtgaaatttaactggtacgttgatggtgtggaagtccataatgccaagaccaagcctagagaggagcaatacaacagtacatatcgcgtggtaagcgtgttgaccgttctccaccaggactggctcaatgggaaagaatacaagtgtaaagtgtccaacaaagctctgccagcacccatcgagaagactatttctaaggccaaaggccagccccgggagcctcaggtctatacacttccaccctcaagggatgaactgaccaagaaccaagtgagcttgacttgcctggtaaaggggttctacccttccgacatcgctgtggagtgggagtctaatggacaaccagaaaacaattacaaaaccacaccccctgtcctcgacagtgatggcagctttttcctgtatagcaaacttaccgttgacaagtccagatggcagcagggaaacgtgttctcatgtagcgtcatgcacgaagctttgcataaccactacacacagaaaagcctcagcctgagtccagggaag

SEQ ID NO: 70 - DNA, 639 bp, Chimeric
gacatccaaatgacccagtcacctagtagcctctccgcctctgttggcgacagggtgacaattacatgcagagcttcacagggtatcaacaattacctgaactggtatcagcagaaaccagggaaggcccccaagcgcttgatatataacaccaataacctgcaaactggcgtccctagccggttctccggatctggtagtggcaccgaatttacactcaccatcagctccctgcagccagaggatttcgccacatactattgtcttcagcataattctttccccacctttgggcaaggaactaaactggagattaagcgtactgtcgccgctccctctgtgttcatttttcctccaagtgatgagcagctcaaaagcggtaccgcatccgttgtgtgcctgcttaacaacttctatccccgggaagccaaggtccaatggaaggtggacaatgctctgcagtcaggaaacagtcaggagagcgtaaccgagcaggattccaaagactctacttactcattgagctccaccctgacactctctaaggcagactatgaaaagcataaagtgtacgcctgtgaggttacccaccagggcctgagtagccctgtgacaaagtccttcaataggggagagtgc

SEQ ID NO: 71 - DNA, 1476 bp, Chimeric
gaggttcagctggagcagtcaggacctgtgctggtgaagcctgggacttcagtgaagatgtcctgtaaggcttctggatacacattcactgactactatataaactggataatacagagccatggaaagtgtcttgagtggattggagttattaatcctgacagcggtggtactgactacaaccagaacttcaagggcaaggccacattgactgttgacaagtcctccaccacagcctacatggaactcactagcctgacatctgaggactctgcagtctattattgtgcaagaagggattcttacggctttgactactggggccaaggcaccactctcacagtctcctcaggcggaggtggctcagggggaggcggtagcggcggaggtggctcagggggaggcggtagcgacattgtgctgacccagactcccaaattcctgcttgtgccagcaggagacaggattaccatgacctgcaaggccagtctgagtgtgactaatgatgtagcttggtatcaacagaaaccagggcagtctcctaaactgctgttatactatgcatccaatcgcaacgctggagtccctgatcgcttcactggcagtggatatgggacggatttcactttcaccatcaccactttgcaggctgaagacctggcagtttatttctgtcagcaggattatacctctcctccgacgttcggttgtggcaccaagctagaaatccgtggtggcggcggttctggcggagggggttctggccccctggggctatggagccagggtggcggcggttctggcggagggggttctggcggtggtggctctggcggtgacatccaaatgacccagtcacctagtagcctctccgcctctgttggcgacagggtgacaattacatgcagagcttcacagggtatcaacaattacctgaactggtatcagcagaaaccagggaaggcccccaagcgcttgatatataacaccaataacctgcaaactggcgtccctagccggttctccggatctggtagtggcaccgaatttacactcaccatcagctccctgcagccagaggatttcgccacatactattgtcttcagcataattctttccccacctttgggcaaggaactaaactggagattaagcgtactgtcgccgctccctctgtgttcatttttcctccaagtgatgagcagctcaaaagcggtaccgcatccgttgtgtgcctgcttaacaacttctatccccgggaagccaaggtccaatggaaggtggacaatgctctgcagtcaggaaacagtcaggagagcgtaaccgagcaggattccaaagactctacttactcattgagctccaccctgacactctctaaggcagactatgaaaagcataaagtgtacgcctgtgaggttacccaccagggcctgagtagccctgtgacaaagtccttcaataggggagagtgc

SEQ ID NO: 72 - protein, 971 aa, Chimeric
QVQLKESGPGLVAPSQSLSITCTVSGFSLTSYGVSWVRQPPGKCLEWLGIIWGDGSTNYHSALISRLSISKDNSKSQVFLKLNSLQTDDTATYYCAKGITTVVDDYYAMDYWGQGTSVTVSSGGGGSGGGGSGGGGSGGGGSDIQMTQSPASLSASVGETVTITCRASENIDSYLAWYQQKQGKSPQLLVYAATFLADDVPSRFSGSGSGTQYSLKINSLQSEDVARYYCQHYYSTPYTFGCGTKLEIKGGGGSVHMPLGFLGPRQARVVNGGGGGSGGGGSEVQLLESGGGLVQPGGSLRLSCAASGFTFSTYAMNWVRQAPGKGLEWVSRIRSKYNNYATYYADSVKGRFTISRDDSKNTLYLQMNSLRAEDTAVYYCVRHGNFGNSYVSWFAYWGQGTLVTVSSASTKGPSVFPLAPSSKSTSGGTAALGCLVKDYFPEPVTVSWNSGALTSGVHTFPAVLQSSGLYSLSSVVTVPSSSLGTQTYICNVNHKPSNTKVDKKVEPKSCDGGGGSGGGGSEVQLVESGGGLVKPGGSLRLSCAASGFTFSNAWMSWVRQAPGKGLEWVGRIKSKTDGGTTDYAAPVKGRFTISRDDSKNTLYLQMNSLKTEDTAVYYCTTPWEWSWYDYWGQGTLVTVSSASTKGPSVFPLAPSSKSTSGGTAALGCLVKDYFPEPVTVSWNSGALTSGVHTFPAVLQSSGLYSLSSVVTVPSSSLGTQTYICNVNHKPSNTKVDKKVEPKSCDKTHTCPPCPAPEAAGGPSVFLFPPKPKDTLMISRTPEVTCVVVDVSHEDPEVKFNWYVDGVEVHNAKTKPREEQYNSTYRVVSVLTVLHQDWLNGKEYKCKVSNKALGAPIEKTISKAKGQPREPQVYTLPPCRDELTKNQVSLWCLVKGFYPSDIAVEWESNGQPENNYKTTPPVLDSDGSFFLYSKLTVDKSRWQQGNVFSCSVMHEALHNHYTQKSLSLSPGK

SEQ ID NO: 73 - protein, 689 aa, Chimeric
EVQLVESGGGLVKPGGSLRLSCAASGFTFSNAWMSWVRQAPGKGLEWVGRIKSKTDGGTTDYAAPVKGRFTISRDDSKNTLYLQMNSLKTEDTAVYYCTTPWEWSWYDYWGQGTLVTVSSASTKGPSVFPLAPSSKSTSGGTAALGCLVKDYFPEPVTVSWNSGALTSGVHTFPAVLQSSGLYSLSSVVTVPSSSLGTQTYICNVNHKPSNTKVDKKVEPKSCDGGGGSGGGGSEVQLLESGGGLVQPGGSLRLSCAASGFTFSTYAMNWVRQAPGKGLEWVSRIRSKYNNYATYYADSVKGRFTISRDDSKNTLYLQMNSLRAEDTAVYYCVRHGNFGNSYVSWFAYWGQGTLVTVSSASTKGPSVFPLAPSSKSTSGGTAALGCLVKDYFPEPVTVSWNSGALTSGVHTFPAVLQSSGLYSLSSVVTVPSSSLGTQTYICNVNHKPSNTKVDKKVEPKSCDKTHTCPPCPAPEAAGGPSVFLFPPKPKDTLMISRTPEVTCVVVDVSHEDPEVKFNWYVDGVEVHNAKTKPREEQYNSTYRVVSVLTVLHQDWLNGKEYKCKVSNKALGAPIEKTISKAKGQPREPQVYTLPPCRDELTKNQVSLWCLVKGFYPSDIAVEWESNGQPENNYKTTPPVLDSDGSFFLYSKLTVDKSRWQQGNVFSCSVMHEALHNHYTQKSLSLSPGK

SEQ ID NO: 74 - protein, 497 aa, Chimeric
QVQLKESGPGLVAPSQSLSITCTVSGFSLTSYGVSWVRQPPGKCLEWLGIIWGDGSTNYHSALISRLSISKDNSKSQVFLKLNSLQTDDTATYYCAKGITTVVDDYYAMDYWGQGTSVTVSSGGGGSGGGGSGGGGSGGGGSDIQMTQSPASLSASVGETVTITCRASENIDSYLAWYQQKQGKSPQLLVYAATFLADDVPSRFSGSGSGTQYSLKINSLQSEDVARYYCQHYYSTPYTFGCGTKLEIKGGGGSGGGGSRQARVVNGGGGGSGGGGSGGGGSQAVVTQEPSLTVSPGGTVTLTCGSSTGAVTTSNYANWVQEKPGQAFRGLIGGTNKRAPGTPARFSGSLLGGKAALTLSGAQPEDEAEYYCALWYSNLWVFGGGTKLTVLGQPKAAPSVTLFPPSSEELQANKATLVCLISDFYPGAVTVAWKADSSPVKAGVETTTPSKQSNNKYAASSYLSLTPEQWKSHRSYSCQVTHEGSTVEKTVAPTECS

SEQ ID NO: 75 - protein, 497 aa, Chimeric
QVQLKESGPGLVAPSQSLSITCTVSGFSLTSYGVSWVRQPPGKCLEWLGIIWGDGSTNYHSALISRLSISKDNSKSQVFLKLNSLQTDDTATYYCAKGITTVVDDYYAMDYWGQGTSVTVSSGGGGSGGGGSGGGGSGGGGSDIQMTQSPASLSASVGETVTITCRASENIDSYLAWYQQKQGKSPQLLVYAATFLADDVPSRFSGSGSGTQYSLKINSLQSEDVARYYCQHYYSTPYTFGCGTKLEIKGGGGSGGGGSGGGGSGGGGGGGSGGGGSGGGGSQAVVTQEPSLTVSPGGTVTLTCGSSTGAVTTSNYANWVQEKPGQAFRGLIGGTNKRAPGTPARFSGSLLGGKAALTLSGAQPEDEAEYYCALWYSNLWVFGGGTKLTVLGQPKAAPSVTLFPPSSEELQANKATLVCLISDFYPGAVTVAWKADSSPVKAGVETTTPSKQSNNKYAASSYLSLTPEQWKSHRSYSCQVTHEGSTVEKTVAPTECS

SEQ ID NO: 76 - protein, 674 aa, Chimeric
QVQLVQSGAEVKKPGASVKVSCKASGYSFTGYTMNWVRQAPGQGLEWMGLITPYNGASSYNQKFRGKATMTVDTSTSTVYMELSSLRSEDTAVYYCARGGYDGRGFDYWGQGTLVTVSSASTKGPSVFPLAPSSKSTSGGTAALGCLVEDYFPEPVTVSWNSGALTSGVHTFPAVLQSSGLYSLSSVVTVPSSSLGTQTYICNVNHKPSNTKVDEKVEPKSCDGGGGSGGGGSQAVVTQEPSLTVSPGGTVTLTCGSSTGAVTTSNYANWVQEKPGQAFRGLIGGTNKRAPGTPARFSGSLLGGKAALTLSGAQPEDEAEYYCALWYSNLWVFGGGTKLTVLSSASTKGPSVFPLAPSSKSTSGGTAALGCLVKDYFPEPVTVSWNSGALTSGVHTFPAVLQSSGLYSLSSVVTVPSSSLGTQTYICNVNHKPSNTKVDKKVEPKSCDKTHTCPPCPAPEAAGGPSVFLFPPKPKDTLMISRTPEVTCVVVDVSHEDPEVKFNWYVDGVEVHNAKTKPREEQYNSTYRVVSVLTVLHQDWLNGKEYKCKVSNKALGAPIEKTISKAKGQPREPQVYTLPPCRDELTKNQVSLWCLVKGFYPSDIAVEWESNGQPENNYKTTPPVLDSDGSFFLYSKLTVDKSRWQQGNVFSCSVMHEALHNHYTQKSLSLSPGK

SEQ ID NO: 77 - protein, 449 aa, Chimeric
QVQLVQSGAEVKKPGASVKVSCKASGYSFTGYTMNWVRQAPGQGLEWMGLITPYNGASSYNQKFRGKATMTVDTSTSTVYMELSSLRSEDTAVYYCARGGYDGRGFDYWGQGTLVTVSSASTKGPSVFPLAPSSKSTSGGTAALGCLVEDYFPEPVTVSWNSGALTSGVHTFPAVLQSSGLYSLSSVVTVPSSSLGTQTYICNVNHKPSNTKVDEKVEPKSCDKTHTCPPCPAPEAAGGPSVFLFPPKPKDTLMISRTPEVTCVVVDVSHEDPEVKFNWYVDGVEVHNAKTKPREEQYNSTYRVVSVLTVLHQDWLNGKEYKCKVSNKALGAPIEKTISKAKGQPREPQVCTLPPSRDELTKNQVSLSCAVKGFYPSDIAVEWESNGQPENNYKTTPPVLDSDGSFFLVSKLTVDKSRWQQGNVFSCSVMHEALHNHYTQKSLSLSPGK

SEQ ID NO: 78 - protein, 213 aa, Chimeric
DIQMTQSPSSLSASVGDRVTITCSASSSVSYMHWYQQKSGKAPKLLIYDTSKLASGVPSRFSGSGSGTDFTLTISSLQPEDFATYYCQQWSKHPLTFGQGTKLEIKRTVAAPSVFIFPPSDRKLKSGTASVVCLLNNFYPREAKVQWKVDNALQSGNSQESVTEQDSKDSTYSLSSTLTLSKADYEKHKVYACEVTHQGLSSPVTKSFNRGEC

SEQ ID NO: 79 - protein, 514 aa, Chimeric
QVQLKESGPGLVAPSQSLSITCTVSGFSLTSYGVSWVRQPPGKCLEWLGIIWGDGSTNYHSALISRLSISKDNSKSQVFLKLNSLQTDDTATYYCAKGITTVVDDYYAMDYWGQGTSVTVSSGGGGSGGGGSGGGGSGGGGSDIQMTQSPASLSASVGETVTITCRASENIDSYLAWYQQKQGKSPQLLVYAATFLADDVPSRFSGSGSGTQYSLKINSLQSEDVARYYCQHYYSTPYTFGCGTKLEIKGGGGSVHMPLGFLGPRQARVVNGGGGGSGGGGSEVQLLESGGGLVQPGGSLRLSCAASGFTFSTYAMNWVRQAPGKGLEWVSRIRSKYNNYATYYADSVKGRFTISRDDSKNTLYLQMNSLRAEDTAVYYCVRHGNFGNSYVSWFAYWGQGTLVTVSSASVAAPSVFIFPPSDEQLKSGTASVVCLLNNFYPREAKVQWKVDNALQSGNSQESVTEQDSKDSTYSLSSTLTLSKADYEKHKVYACEVTHQGLSSPVTKSFNRGEC

SEQ ID NO: 80 - protein, 514 aa, Chimeric
QVQLKESGPGLVAPSQSLSITCTVSGFSLTSYGVSWVRQPPGKCLEWLGIIWGDGSTNYHSALISRLSISKDNSKSQVFLKLNSLQTDDTATYYCAKGITTVVDDYYAMDYWGQGTSVTVSSGGGGSGGGGSGGGGSGGGGSDIQMTQSPASLSASVGETVTITCRASENIDSYLAWYQQKQGKSPQLLVYAATFLADDVPSRFSGSGSGTQYSLKINSLQSEDVARYYCQHYYSTPYTFGCGTKLEIKGGGGSGGGGSGGGGSGGGGGGGSGGGGSGGGGSEVQLLESGGGLVQPGGSLRLSCAASGFTFSTYAMNWVRQAPGKGLEWVSRIRSKYNNYATYYADSVKGRFTISRDDSKNTLYLQMNSLRAEDTAVYYCVRHGNFGNSYVSWFAYWGQGTLVTVSSASVAAPSVFIFPPSDEQLKSGTASVVCLLNNFYPREAKVQWKVDNALQSGNSQESVTEQDSKDSTYSLSSTLTLSKADYEKHKVYACEVTHQGLSSPVTKSFNRGEC

SEQ ID NO: 81 - protein, 232 aa, Chimeric
EVQLLESGGGLVQPGGSLRLSCAASGFTFSTYAMNWVRQAPGKGLEWVSRIRSKYNNYATYYADSVKGRFTISRDDSKNTLYLQMNSLRAEDTAVYYCVRHGNFGNSYVSWFAYWGQGTLVTVSSASVAAPSVFIFPPSDEQLKSGTASVVCLLNNFYPREAKVQWKVDNALQSGNSQESVTEQDSKDSTYSLSSTLTLSKADYEKHKVYACEVTHQGLSSPVTKSFNRGEC

SEQ ID NO: 82 - protein, 956 aa, Chimeric
QVQLKESGPGLVAPSQSLSITCTVSGFSLTSYGVSWVRQPPGKCLEWLGIIWGDGSTNYHSALISRLSISKDNSKSQVFLKLNSLQTDDTATYYCAKGITTVVDDYYAMDYWGQGTSVTVSSGGGGSGGGGSGGGGSGGGGSDIQMTQSPASLSASVGETVTITCRASENIDSYLAWYQQKQGKSPQLLVYAATFLADDVPSRFSGSGSGTQYSLKINSLQSEDVARYYCQHYYSTPYTFGCGTKLEIKGGGGSVHMPLGFLGPRQARVVNGGGGGSGGGGSQAVVTQEPSLTVSPGGTVTLTCGSSTGAVTTSNYANWVQEKPGQAFRGLIGGTNKRAPGTPARFSGSLLGGKAALTLSGAQPEDEAEYYCALWYSNLWVFGGGTKLTVLSSASTKGPSVFPLAPSSKSTSGGTAALGCLVKDYFPEPVTVSWNSGALTSGVHTFPAVLQSSGLYSLSSVVTVPSSSLGTQTYICNVNHKPSNTKVDKKVEPKSCDGGGGSGGGGSQVQLVQSGAEVKKPGASVKVSCKASGYSFTGYTMNWVRQAPGQGLEWMGLITPYNGASSYNQKFRGKATMTVDTSTSTVYMELSSLRSEDTAVYYCARGGYDGRGFDYWGQGTLVTVSSASTKGPSVFPLAPSSKSTSGGTAALGCLVEDYFPEPVTVSWNSGALTSGVHTFPAVLQSSGLYSLSSVVTVPSSSLGTQTYICNVNHKPSNTKVDEKVEPKSCDKTHTCPPCPAPEAAGGPSVFLFPPKPKDTLMISRTPEVTCVVVDVSHEDPEVKFNWYVDGVEVHNAKTKPREEQYNSTYRVVSVLTVLHQDWLNGKEYKCKVSNKALGAPIEKTISKAKGQPREPQVYTLPPCRDELTKNQVSLWCLVKGFYPSDIAVEWESNGQPENNYKTTPPVLDSDGSFFLYSKLTVDKSRWQQGNVFSCSVMHEALHNHYTQKSLSLSPGK

SEQ ID NO: 83 - protein, 956 aa, Chimeric
QVQLKESGPGLVAPSQSLSITCTVSGFSLTSYGVSWVRQPPGKCLEWLGIIWGDGSTNYHSALISRLSISKDNSKSQVFLKLNSLQTDDTATYYCAKGITTVVDDYYAMDYWGQGTSVTVSSGGGGSGGGGSGGGGSGGGGSDIQMTQSPASLSASVGETVTITCRASENIDSYLAWYQQKQGKSPQLLVYAATFLADDVPSRFSGSGSGTQYSLKINSLQSEDVARYYCQHYYSTPYTFGCGTKLEIKGGGGSGGGGSGGGGSGGGGGGGSGGGGSGGGGSQAVVTQEPSLTVSPGGTVTLTCGSSTGAVTTSNYANWVQEKPGQAFRGLIGGTNKRAPGTPARFSGSLLGGKAALTLSGAQPEDEAEYYCALWYSNLWVFGGGTKLTVLSSASTKGPSVFPLAPSSKSTSGGTAALGCLVKDYFPEPVTVSWNSGALTSGVHTFPAVLQSSGLYSLSSVVTVPSSSLGTQTYICNVNHKPSNTKVDKKVEPKSCDGGGGSGGGGSQVQLVQSGAEVKKPGASVKVSCKASGYSFTGYTMNWVRQAPGQGLEWMGLITPYNGASSYNQKFRGKATMTVDTSTSTVYMELSSLRSEDTAVYYCARGGYDGRGFDYWGQGTLVTVSSASTKGPSVFPLAPSSKSTSGGTAALGCLVEDYFPEPVTVSWNSGALTSGVHTFPAVLQSSGLYSLSSVVTVPSSSLGTQTYICNVNHKPSNTKVDEKVEPKSCDKTHTCPPCPAPEAAGGPSVFLFPPKPKDTLMISRTPEVTCVVVDVSHEDPEVKFNWYVDGVEVHNAKTKPREEQYNSTYRVVSVLTVLHQDWLNGKEYKCKVSNKALGAPIEKTISKAKGQPREPQVYTLPPCRDELTKNQVSLWCLVKGFYPSDIAVEWESNGQPENNYKTTPPVLDSDGSFFLYSKLTVDKSRWQQGNVFSCSVMHEALHNHYTQKSLSLSPGK

SEQ ID NO: 84 - protein, 674 aa, Chimeric
QAVVTQEPSLTVSPGGTVTLTCGSSTGAVTTSNYANWVQEKPGQAFRGLIGGTNKRAPGTPARFSGSLLGGKAALTLSGAQPEDEAEYYCALWYSNLWVFGGGTKLTVLSSASTKGPSVFPLAPSSKSTSGGTAALGCLVKDYFPEPVTVSWNSGALTSGVHTFPAVLQSSGLYSLSSVVTVPSSSLGTQTYICNVNHKPSNTKVDKKVEPKSCDGGGGSGGGGSQVQLVQSGAEVKKPGASVKVSCKASGYSFTGYTMNWVRQAPGQGLEWMGLITPYNGASSYNQKFRGKATMTVDTSTSTVYMELSSLRSEDTAVYYCARGGYDGRGFDYWGQGTLVTVSSASTKGPSVFPLAPSSKSTSGGTAALGCLVEDYFPEPVTVSWNSGALTSGVHTFPAVLQSSGLYSLSSVVTVPSSSLGTQTYICNVNHKPSNTKVDEKVEPKSCDKTHTCPPCPAPEAAGGPSVFLFPPKPKDTLMISRTPEVTCVVVDVSHEDPEVKFNWYVDGVEVHNAKTKPREEQYNSTYRVVSVLTVLHQDWLNGKEYKCKVSNKALGAPIEKTISKAKGQPREPQVYTLPPCRDELTKNQVSLWCLVKGFYPSDIAVEWESNGQPENNYKTTPPVLDSDGSFFLYSKLTVDKSRWQQGNVFSCSVMHEALHNHYTQKSLSLSPGK

SEQ ID NO: 85 - protein, 971 aa, Chimeric
QVQLKESGPGLVAPSQSLSITCTVSGFSLTSYGVSWVRQPPGKCLEWLGIIWGDGSTNYHSALISRLSISKDNSKSQVFLKLNSLQTDDTATYYCAKGITTVVDDYYAMDYWGQGTSVTVSSGGGGSGGGGSGGGGSGGGGSDIQMTQSPASLSASVGETVTITCRASENIDSYLAWYQQKQGKSPQLLVYAATFLADDVPSRFSGSGSGTQYSLKINSLQSEDVARYYCQHYYSTPYTFGCGTKLEIKGGGGSGGGGSGGGGSFVGGTGGGGSGGGGSGGSEVQLLESGGGLVQPGGSLRLSCAASGFTFSTYAMNWVRQAPGKGLEWVSRIRSKYNNYATYYADSVKGRFTISRDDSKNTLYLQMNSLRAEDTAVYYCVRHGNFGNSYVSWFAYWGQGTLVTVSSASTKGPSVFPLAPSSKSTSGGTAALGCLVKDYFPEPVTVSWNSGALTSGVHTFPAVLQSSGLYSLSSVVTVPSSSLGTQTYICNVNHKPSNTKVDKKVEPKSCDGGGGSGGGGSEVQLVESGGGLVKPGGSLRLSCAASGFTFSNAWMSWVRQAPGKGLEWVGRIKSKTDGGTTDYAAPVKGRFTISRDDSKNTLYLQMNSLKTEDTAVYYCTTPWEWSWYDYWGQGTLVTVSSASTKGPSVFPLAPSSKSTSGGTAALGCLVKDYFPEPVTVSWNSGALTSGVHTFPAVLQSSGLYSLSSVVTVPSSSLGTQTYICNVNHKPSNTKVDKKVEPKSCDKTHTCPPCPAPEAAGGPSVFLFPPKPKDTLMISRTPEVTCVVVDVSHEDPEVKFNWYVDGVEVHNAKTKPREEQYNSTYRVVSVLTVLHQDWLNGKEYKCKVSNKALGAPIEKTISKAKGQPREPQVYTLPPCRDELTKNQVSLWCLVKGFYPSDIAVEWESNGQPENNYKTTPPVLDSDGSFFLYSKLTVDKSRWQQGNVFSCSVMHEALHNHYTQKSLSLSPGK

SEQ ID NO: 86 - protein, 33 aa, Chimeric
GGGGSVHMPLGFLGPRQARVVNGGGGGSGGGGS

SEQ ID NO: 87 - protein, 35 aa, Chimeric
GGGGSVHMPLGFLGPRQARVVNGGGGGSGGGGSGG

SEQ ID NO: 88 - protein, 33 aa, Chimeric
GGGGSGGGGSGGGGSFVGGTGGGGSGGGGSGGS

SEQ ID NO: 89 - protein, 33 aa, Chimeric
GGGGSGGGGSKKAAPVNGGGGGSGGGGSGGGGS

SEQ ID NO: 90 - protein, 33 aa, Chimeric
GGGGSGGGGSPMAKKVNGGGGGSGGGGSGGGGS

SEQ ID NO: 91 - protein, 33 aa, Chimeric
GGGGSGGGGSQARAKVNGGGGGSGGGGSGGGGS

SEQ ID NO: 92 - protein, 33 aa, Chimeric
GGGGSGGGGSVHMPLGFLGPGGGGSGGGGSGGS

SEQ ID NO: 93 - protein, 33 aa, Chimeric
GGGGSGGGGSQARAKGGGGSGGGGSGGGGSGGS

SEQ ID NO: 94 - protein, 33 aa, Chimeric
GGGGSVHMPLGFLGPPMAKKGGGGSGGGGSGGS

SEQ ID NO: 95 - protein, 33 aa, Chimeric
GGGGSGGGGSKKAAPGGGGSGGGGSGGGGSGGS

SEQ ID NO: 96 - protein, 33 aa, Chimeric
GGGGSGGGGSPMAKKGGGGSGGGGSGGGGSGGS

SEQ ID NO: 97 - protein, 18 aa, Chimeric
VHMPLGFLGPRQARVVNG

SEQ ID NO: 98 - protein, 6 aa, Chimeric
FVGGTG

SEQ ID NO: 99 - protein, 8 aa, Chimeric
KKAAPVNG

SEQ ID NO: 100 - protein, 8 aa, Chimeric
PMAKKVNG

SEQ ID NO: 101 - protein, 8 aa, Chimeric
QARAKVNG

SEQ ID NO: 102 - protein, 10 aa, Chimeric
VHMPLGFLGP

SEQ ID NO: 103 - protein, 5 aa, Chimeric
QARAK

SEQ ID NO: 104 - protein, 15 aa, Chimeric
VHMPLGFLGPPMAKK

SEQ ID NO: 105 - protein, 5 aa, Chimeric
KKAAP

SEQ ID NO: 106 - protein, 5 aa, Chimeric
PMAKK

SEQ ID NO: 107 - protein, 5 aa, Chimeric
GYTMN

SEQ ID NO: 108 - protein, 17 aa, Chimeric
LITPYNGASSYNQKFRG

SEQ ID NO: 109 - protein, 10 aa, Chimeric
GGYDGRGFDY

SEQ ID NO: 110 - protein, 10 aa, Chimeric
SASSSVSYMH

SEQ ID NO: 111 - protein, 7 aa, Chimeric
DTSKLAS

SEQ ID NO: 112 - protein, 9 aa, Chimeric
QQWSKHPLT

SEQ ID NO: 113 - protein, 119 aa, Chimeric
QVQLVQSGAEVKKPGASVKVSCKASGYSFTGYTMNWVRQAPGQGLEWMGLITPYNGASSYNQKFRGKATMTVDTSTSTVYMELSSLRSEDTAVYYCARGGYDGRGFDYWGQGTLVTVSS

SEQ ID NO: 114 - protein, 106 aa, Chimeric
DIQMTQSPSSLSASVGDRVTITCSASSSVSYMHWYQQKSGKAPKLLIYDTSKLASGVPSRFSGSGSGTDFTLTISSLQPEDFATYYCQQWSKHPLTFGQGTKLEIK

SEQ ID NO: 115 - protein, 120 aa, Chimeric [sequence omitted]

SEQ ID NO: 116 - protein, 106 aa, Chimeric [sequence omitted]

SEQ ID NO: 117 - DNA, 648 bp, Chimeric; identical to SEQ ID NO: 62

SEQ ID NO: 118 - DNA, 2916 bp, Chimeric
caagtgcagctgaaagagtccggccctggactggtggcccctagccagagcctgagcatcacctgtaccgtgtccggcttcagcctgaccagctacggcgtgtcatgggtgcgccagcctccaggcaagtgtctggaatggctgggcatcatctggggcgacggcagcaccaattaccacagcgccctgatcagcagactgagcatctccaaggacaacagcaagagccaggtgttcctgaagctgaacagcctgcagaccgacgacaccgccacctactactgcgccaagggcatcaccaccgtggtggacgactactacgctatggactactggggccagggcaccagcgtgacagtgtctagcggaggcggaggatctggcggcggaggaagtggcggagggggatctgggggaggcggaagcgatatccagatgacccagagccctgccagcctgtctgcctctgtgggcgagacagtgaccatcacatgccgggccagcgagaacatcgacagctacctggcctggtatcagcagaagcagggcaagagcccccagctgctggtgtacgccgccacctttctggccgacgatgtgcccagcagattcagcggcagcggaagcggcacacagtacagcctgaagatcaactccctgcagagcgaggacgtggcccggtactactgccagcactactacagcaccccctacaccttcggctgcggcaccaagctggaaatcaaaggaggcggcggaagtgtgcacatgcccctgggcttcctgggccccagacaggccagagtcgtgaacggggggggcggaggcagtggggggggaggatccgaggtgcagctgctggaatctggcggcggactggtgcagcctggcggatctctgagactgagctgtgccgccagcggcttcaccttcagcacctacgccatgaactgggtgcgccaggcccctggcaaaggcctggaatgggtgtcccggatcagaagcaagtacaacaactacgccacctactacgccgacagcgtgaagggccggttcaccatcagccgggacgacagcaagaacaccctgtacctgcagatgaacagcctgcgggccgaggacaccgccgtgtactattgtgtgcggcacggcaacttcggcaacagctatgtgtcttggtttgcctactggggccagggcaccctcgtgaccgtgtcaagcgctagcacaaagggccctagcgtgttccctctggcccccagcagcaagagcacaagcggcggaacagccgccctgggctgcctcgtgaaggactacttccccgagcccgtgacagtgtcttggaacagcggagccctgacaagcggcgtgcacaccttccctgccgtgctgcagagcagcggcctgtactccctgagcagcgtggtcaccgtgcctagcagcagcctgggcacccagacctacatctgcaacgtgaaccacaagcccagcaacaccaaagtggacaagaaggtggagcccaagagctgtgatggcggaggagggtccgggggcggaggatccgaggtgcaattggttgaatctggtggtggtctggtaaaaccgggcggttccctgcgtctgagctgcgcggcttccgggttcaccttctccaacgcgtggatgagctgggttcgccaggccccgggcaaaggcctcgagtgggttggtcgtatcaagtctaaaactgacggtggcaccacggattacgcggctccagttaaaggtcgttttaccatttcccgcgacgatagcaaaaacactctgtatctgcagatgaactctctgaaaactgaagacaccgcagtctactactgtactaccccgtgggaatggtcttggtacgattattggggccagggcacgctggttacggtgtctagcgctagtaccaagggccccagcgtgttccccctggcacccagcagcaagagcacatctggcggaacagccgctctgggctgtctggtgaaagactacttccccgagcccgtgaccgtgtcttggaactctggcgccctgaccagcggcgtgcacacctttccagccgtgctgcagagcagcggcctgtactccctgtcctccgtggtcaccgtgccctctagctccctgggaacacagacatatatctgtaatgtcaatcacaagccttccaacaccaaagtcgataagaaagtcgagcccaagagctgcgacaaaactcacacatgcccaccgtgcccagcacctgaagctgcagggggaccgtcagtcttcctcttccccccaaaacccaaggacaccctcatgatctcccggacccctgaggtcacatgcgtggtggtggacgtgagccacgaagaccctgaggtcaagttcaactggtacgtggacggcgtggaggtgcataatgccaagacaaagccgcgggaggagcagtacaacagcacgtaccgtgtggtcagcgtcctcaccgtcctgcaccaggactggctgaatggcaaggagtacaagtgcaaggtctccaacaaagccctcggcgcccccatcgagaaaaccatctccaaagccaaagggcagccccgagaaccacaggtgtacaccctgcccccatgccgggatgagctgaccaagaaccaggtcagcctgtggtgcctggtcaaaggcttctatcccagcgacatcgccgtggagtgggagagcaatgggcagccggagaacaactacaagaccacgcctcccgtgctggactccgacggctccttcttcctctacagcaagctcaccgtggacaagagcaggtggcagcaggggaacgtcttctcatgctccgtgatgcatgaggctctgcacaaccactacacgcagaagagcctctccctgtctccgggtaaatga

SEQ ID NO: 119 - DNA, 2070 bp, Chimeric
gaggtgcaattggttgaatctggtggtggtctggtaaaaccgggcggttccctgcgtctgagctgcgcggcttccggattcaccttctccaacgcgtggatgagctgggttcgccaggccccgggcaaaggcctcgagtgggttggtcgtatcaagtctaaaactgacggtggcaccacggattacgcggctccagttaaaggtcgttttaccatttcccgcgacgatagcaaaaacactctgtatctgcagatgaactctctgaaaactgaagacaccgcagtctactactgtactaccccgtgggaatggtcttggtacgattattggggccagggcacgctggttacggtgtcttccgctagcacaaagggccctagcgtgttccctctggcccccagcagcaagagcacaagcggcggaacagccgccctgggctgcctcgtgaaggactacttccccgagcccgtgacagtgtcttggaacagcggagccctgacaagcggcgtgcacactttccctgccgtgctgcagagcagcggcctgtactccctgagcagcgtggtcaccgtgcctagcagcagcctgggcacccagacctacatctgcaacgtgaaccacaagcccagcaacaccaaagtggacaagaaggtggagcccaagagctgtgatggcggaggagggtccggaggcggaggatccgaggtgcagctgctggaatctggcggcggactggtgcagcctggcggatctctgagactgagctgtgccgccagcggcttcaccttcagcacctacgccatgaactgggtgcgccaggcccctggcaaaggcctggaatgggtgtcccggatcagaagcaagtacaacaactacgccacctactacgccgacagcgtgaagggccggttcaccatcagccgggacgacagcaagaacaccctgtacctgcagatgaacagcctgcgggccgaggacaccgccgtgtactattgtgtgcggcacggcaacttcggcaacagctatgtgtcttggtttgcctactggggccagggcaccctcgtgaccgtgtcaagcgctagtaccaagggccccagcgtgttccccctggcacccagcagcaagagcacatctggcggaacagccgctctgggctgtctggtgaaagactacttccccgagcccgtgaccgtgtcttggaactctggcgccctgaccagcggcgtgcacacctttccagccgtgctgcagagcagcggcctgtactccctgtcctccgtggtcaccgtgccctctagctccctgggaacacagacatatatctgtaatgtcaatcacaagccttccaacaccaaagtcgataagaaagtcgagcccaagagctgcgacaaaactcacacatgcccaccgtgcccagcacctgaagctgcagggggaccgtcagtcttcctcttccccccaaaacccaaggacaccctcatgatctcccggacccctgaggtcacatgcgtggtggtggacgtgagccacgaagaccctgaggtcaagttcaactggtacgtggacggcgtggaggtgcataatgccaagacaaagccgcgggaggagcagtacaacagcacgtaccgtgtggtcagcgtcctcaccgtcctgcaccaggactggctgaatggcaaggagtacaagtgcaaggtctccaacaaagccctcggcgcccccatcgagaaaaccatctccaaagccaaagggcagccccgagaaccacaggtgtacaccctgcccccatgccgggatgagctgaccaagaaccaggtcagcctgtggtgcctggtcaaaggcttctatcccagcgacatcgccgtggagtgggagagcaatgggcagccggagaacaactacaagaccacgcctcccgtgctggactccgacggctccttcttcctctacagcaagctcaccgtggacaagagcaggtggcagcaggggaacgtcttctcatgctccgtgatgcatgaggctctgcacaaccactacacgcagaagagcctctccctgtctccgggtaaatga

SEQ ID NO: 120 - DNA, 1494 bp, Chimeric
caagtgcagctgaaagagtccggccctggactggtggcccctagccagagcctgagcatcacctgtaccgtgtccggcttcagcctgaccagctacggcgtgtcatgggtgcgccagcctccaggcaagtgtctggaatggctgggcatcatctggggcgacggcagcaccaattaccacagcgccctgatcagcagactgagcatctccaaggacaacagcaagagccaggtgttcctgaagctgaacagcctgcagaccgacgacaccgccacctactactgcgccaagggcatcaccaccgtggtggacgactactacgctatggactactggggccagggcaccagcgtgacagtgtctagcggaggcggaggatctggcggcggaggaagtggcggagggggatctgggggaggcggaagcgatatccagatgacccagagccctgccagcctgtctgcctctgtgggcgagacagtgaccatcacatgccgggccagcgagaacatcgacagctacctggcctggtatcagcagaagcagggcaagagcccccagctgctggtgtacgccgccacctttctggccgacgatgtgcccagcagattcagcggcagcggaagcggcacacagtacagcctgaagatcaactccctgcagagcgaggacgtggcccggtactactgccagcactactacagcaccccctacaccttcggctgcggcaccaagctggaaatcaaaggcgggggaggctccggaggcggcggaagtagacaggccagagtcgtgaacgggggaggggggggaagtgggggcggaggcagtgggggcggaggatcccaggccgtcgtgacccaggaacccagcctgacagtgtctcctggcggcaccgtgaccctgacatgtggcagttctacaggcgccgtgaccaccagcaactacgccaactgggtgcaggaaaagcccggccaggccttcagaggactgatcggcggcaccaacaagagagcccctggcacccctgccagattcagcggatctctgctgggaggaaaggccgccctgacactgtctggcgcccagccagaagatgaggccgagtactactgcgccctgtggtacagcaacctgtgggtgttcggcggaggcaccaagctgacagtcctaggtcaacccaaggctgcccccagcgtgaccctgttcccccccagcagcgaggaactgcaggccaacaaggccaccctggtctgcctgatcagcgacttctacccaggcgccgtgaccgtggcctggaaggccgacagcagccccgtgaaggccggcgtggagaccaccacccccagcaagcagagcaacaacaagtacgccgccagcagctacctgagcctgacccccgagcagtggaagagccacaggtcctacagctgccaggtgacccacgagggcagcaccgtggagaaaaccgtggcccccaccgagtgcagctga

SEQ ID NO: 121 - DNA, 1494 bp, Chimeric
caagtgcagctgaaagagtccggccctggactggtggcccctagccagagcctgagcatcacctgtaccgtgtccggcttcagcctgaccagctacggcgtgtcatgggtgcgccagcctccaggcaagtgtctggaatggctgggcatcatctggggcgacggcagcaccaattaccacagcgccctgatcagcagactgagcatctccaaggacaacagcaagagccaggtgttcctgaagctgaacagcctgcagaccgacgacaccgccacctactactgcgccaagggcatcaccaccgtggtggacgactactacgctatggactactggggccagggcaccagcgtgacagtgtctagcggaggcggaggatctggcggcggaggaagtggcggagggggatctgggggaggcggaagcgatatccagatgacccagagccctgccagcctgtctgcctctgtgggcgagacagtgaccatcacatgccgggccagcgagaacatcgacagctacctggcctggtatcagcagaagcagggcaagagcccccagctgctggtgtacgccgccacctttctggccgacgatgtgcccagcagattcagcggcagcggaagcggcacacagtacagcctgaagatcaactccctgcagagcgaggacgtggcccggtactactgccagcactactacagcaccccctacaccttcggctgcggcaccaagctggaaatcaaaggcgggggaggctccggaggcggcggaagtggaggcggcggaagtggcggaggcggaggggggggaagtgggggcggaggcagtggggggggaggatcccaggccgtcgtgacccaggaacccagcctgacagtgtctcctggcggcaccgtgaccctgacatgtggcagttctacaggcgccgtgaccaccagcaactacgccaactgggtgcaggaaaagcccggccaggccttcagaggactgatcggcggcaccaacaagagagcccctggcacccctgccagattcagcggatctctgctgggaggaaaggccgccctgacactgtctggcgcccagccagaagatgaggccgagtactactgcgccctgtggtacagcaacctgtgggtgttcggcggaggcaccaagctgacagtcctaggtcaacccaaggctgcccccagcgtgaccctgttcccccccagcagcgaggaactgcaggccaacaaggccaccctggtctgcctgatcagcgacttctacccaggcgccgtgaccgtggcctggaaggccgacagcagccccgtgaaggccggcgtggagaccaccacccccagcaagcagagcaacaacaagtacgccgccagcagctacctgagcctgacccccgagcagtggaagagccacaggtcctacagctgccaggtgacccacgagggcagcaccgtggagaaaaccgtggcccccaccgagtgcagctga

SEQ ID NO: 122 - DNA, 2025 bp, Chimeric
caggtgcagctggtgcagtctggcgccgaagtgaagaaaccaggcgccagcgtgaaggtgtcctgcaaggccagcggctacagcttcaccggctacaccatgaactgggtgcgccaggctcctggacagggcctggaatggatgggcctgatcaccccctacaacggcgccagcagctacaaccagaagttccggggcaaggccaccatgaccgtggacaccagcacctccaccgtgtatatggaactgagcagcctgcggagcgaggacaccgccgtgtactattgtgccagaggcggctacgacggcagaggcttcgattattggggccagggcaccctcgtgaccgtgtcctctgctagcaccaagggcccctccgtgtttcctctggccccttccagcaagtccacctctggcggaactgccgctctgggctgcctggtggaagattacttccccgagcccgtgaccgtgtcctggaattctggcgctctgacctccggcgtgcacacctttccagctgtgctgcagtcctccggcctgtactccctgtcctccgtcgtgacagtgccctccagctctctgggcacccagacctacatctgcaacgtgaaccacaagccctccaacaccaaggtggacgagaaggtggaacccaagtcctgcgacggtggcggaggttccggaggcggaggatcccaggctgtcgtgacccaggaaccctccctgacagtgtctcctggcggcaccgtgaccctgacctgtggatcttctaccggcgctgtgaccacctccaactacgccaattgggtgcaggaaaagcccggccaggccttcagaggactgatcggcggcaccaacaagagagcccctggcacccctgccagattctccggttctctgctgggcggcaaggctgccctgactctgtctggtgctcagcctgaggacgaggccgagtactactgcgccctgtggtactccaacctgtgggtgttcggcggaggcaccaagctgaccgtgctgtccagcgcttccaccaagggacccagtgtgttccccctggcccccagctccaagtctacatccggtggcacagctgccctgggatgtctcgtgaaggactactttcctgagcctgtgacagtgtcttggaacagcggagccctgaccagcggagtgcacacattccctgcagtgctgcagagcagcggcctgtatagcctgagcagcgtcgtgaccgtgccttcctctagcctgggaacacagacatatatctgtaatgtgaatcataagcccagtaataccaaagtggataagaaagtggaacctaagagctgcgataagacccacacctgtcccccctgccctgctcctgaagctgctggtggccctagcgtgttcctgttccccccaaagcccaaggacaccctgatgatctcccggacccccgaagtgacctgcgtggtggtggatgtgtcccacgaggaccctgaagtgaagttcaattggtacgtggacggcgtggaagtgcacaacgccaagaccaagcctagagaggaacagtacaactccacctaccgggtggtgtccgtgctgacagtgctgcaccaggactggctgaacggcaaagagtacaagtgcaaggtgtccaacaaggccctgggcgctcccatcgaaaagaccatctccaaggccaagggccagccccgggaaccccaggtgtacaccctgcccccatgccgggatgagctgaccaagaaccaggtcagcctgtggtgcctggtcaaaggcttctatcccagcgacatcgccgtggagtgggagagcaatgggcagccggagaacaactacaagaccacgcctcccgtgctggactccgacggctccttcttcctctacagcaagctcaccgtggacaagagcaggtggcagcaggggaacgtcttctcatgctccgtgatgcatgaggctctgcacaaccactacacgcagaagagcctctccctgtctccgggtaaatga

SEQ ID NO: 123 - DNA, 1350 bp, Chimeric
caggtgcagctggtgcagtctggcgccgaagtgaagaaaccaggcgccagcgtgaaggtgtcctgcaaggccagcggctacagcttcaccggctacaccatgaactgggtgcgccaggctcctggacagggcctggaatggatgggcctgatcaccccctacaacggcgccagcagctacaaccagaagttccggggcaaggccaccatgaccgtggacaccagcacctccaccgtgtatatggaactgagcagcctgcggagcgaggacaccgccgtgtactattgtgccagaggcggctacgacggcagaggcttcgattattggggccagggcaccctcgtgaccgtgtcctctgctagcaccaagggcccctccgtgttccccctggcccccagcagcaagagcaccagcggcggcacagccgctctgggctgcctggtcgaggactacttccccgagcccgtgaccgtgtcctggaacagcggagccctgacctccggcgtgcacaccttccccgccgtgctgcagagttctggcctgtatagcctgagcagcgtggtcaccgtgccttctagcagcctgggcacccagacctacatctgcaacgtgaaccacaagcccagcaacaccaaggtggacgagaaggtggagcccaagagctgcgacaaaactcacacatgcccaccgtgcccagcacctgaagctgcagggggaccgtcagtcttcctcttccccccaaaacccaaggacaccctcatgatctcccggacccctgaggtcacatgcgtggtggtggacgtgagccacgaagaccctgaggtcaagttcaactggtacgtggacggcgtggaggtgcataatgccaagacaaagccgcgggaggagcagtacaacagcacgtaccgtgtggtcagcgtcctcaccgtcctgcaccaggactggctgaatggcaaggagtacaagtgcaaggtctccaacaaagccctcggcgcccccatcgagaaaaccatctccaaagccaaagggcagccccgagaaccacaggtgtgcaccctgcccccatcccgggatgagctgaccaagaaccaggtcagcctctcgtgcgcagtcaaaggcttctatcccagcgacatcgccgtggagtgggagagcaatgggcagccggagaacaactacaagaccacgcctcccgtgctggactccgacggctccttcttcctcgtgagcaagctcaccgtggacaagagcaggtggcagcaggggaacgtcttctcatgctccgtgatgcatgaggctctgcacaaccactacacgcagaagagcctctccctgtctccgggtaaatga

SEQ ID NO: 124 - DNA, 642 bp, Chimeric
gacatccagatgacccagagccccagcagcctgtctgccagcgtgggcgacagagtgaccatcacctgtagcgccagcagcagcgtgtcctacatgcactggtatcagcagaagtccggcaaggcccccaagctgctgatctacgacaccagcaagctggcctccggcgtgcccagcagattttctggcagcggctccggcaccgacttcaccctgacaatcagctccctccagcccgaggacttcgccacctactactgccagcagtggtccaagcaccccctgacctttggccagggcaccaagctggaaatcaagcgtacggtggctgcaccatctgtcttcatcttcccgccatctgatcggaagttgaaatctggaactgcctctgttgtgtgcctgctgaataacttctatcccagagaggccaaagtacagtggaaggtggataacgccctccaatcgggtaactcccaggagagtgtcacagagcaggacagcaaggacagcacctacagcctcagcagcaccctgacgctgagcaaagcagactacgagaaacacaaagtctacgcctgcgaagtcacccatcagggcctgagctcgcccgtcacaaagagcttcaacaggggagagtgttag

SEQ ID NO: 125 - DNA, 1545 bp, Chimeric
caagtgcagctgaaagagtccggccctggactggtggcccctagccagagcctgagcatcacctgtaccgtgtccggcttcagcctgaccagctacggcgtgtcatgggtgcgccagcctccaggcaagtgtctggaatggctgggcatcatctggggcgacggcagcaccaattaccacagcgccctgatcagcagactgagcatctccaaggacaacagcaagagccaggtgttcctgaagctgaacagcctgcagaccgacgacaccgccacctactactgcgccaagggcatcaccaccgtggtggacgactactacgctatggactactggggccagggcaccagcgtgacagtgtctagcggaggcggaggatctggcggcggaggaagtggcggagggggatctgggggaggcggaagcgatatccagatgacccagagccctgccagcctgtctgcctctgtgggcgagacagtgaccatcacatgccgggccagcgagaacatcgacagctacctggcctggtatcagcagaagcagggcaagagcccccagctgctggtgtacgccgccacctttctggccgacgatgtgcccagcagattcagcggcagcggaagcggcacacagtacagcctgaagatcaactccctgcagagcgaggacgtggcccggtactactgccagcactactacagcaccccctacaccttcggctgcggcaccaagctggaaatcaaaggaggcggcggaagtgtgcacatgcccctgggcttcctgggccccagacaggccagagtcgtgaacggggggggcggaggcagtggggggggaggatccgaggtgcagctgctggaatctggcggcggactggtgcagcctggcggatctctgagactgagctgtgccgccagcggcttcaccttcagcacctacgccatgaactgggtgcgccaggcccctggcaaaggcctggaatgggtgtcccggatcagaagcaagtacaacaactacgccacctactacgccgacagcgtgaagggccggttcaccatcagccgggacgacagcaagaacaccctgtacctgcagatgaacagcctgcgggccgaggacaccgccgtgtactattgtgtgcggcacggcaacttcggcaacagctatgtgtcttggtttgcctactggggccagggcaccctcgtgaccgtgtcaagcgctagcgtggccgctccctccgtgttcatcttcccaccttccgacgagcagctgaagtccggcaccgcttctgtcgtgtgcctgctgaacaacttctacccccgcgaggccaaggtgcagtggaaggtggacaacgccctgcagtccggcaacagccaggaatccgtgaccgagcaggactccaaggacagcacctactccctgtcctccaccctgaccctgtccaaggccgactacgagaagcacaaggtgtacgcctgcgaagtgacccaccagggcctgtctagccccgtgaccaagtctttcaaccggggcgagtgctga

SEQ ID NO: 126 - DNA, 1545 bp, Chimeric
caagtgcagctgaaagagtccggccctggactggtggcccctagccagagcctgagcatcacctgtaccgtgtccggcttcagcctgaccagctacggcgtgtcatgggtgcgccagcctccaggcaagtgtctggaatggctgggcatcatctggggcgacggcagcaccaattaccacagcgccctgatcagcagactgagcatctccaaggacaacagcaagagccaggtgttcctgaagctgaacagcctgcagaccgacgacaccgccacctactactgcgccaagggcatcaccaccgtggtggacgactactacgctatggactactggggccagggcaccagcgtgacagtgtctagcggaggcggaggatctggcggcggaggaagtggcggagggggatctgggggaggcggaagcgatatccagatgacccagagccctgccagcctgtctgcctctgtgggcgagacagtgaccatcacatgccgggccagcgagaacatcgacagctacctggcctggtatcagcagaagcagggcaagagcccccagctgctggtgtacgccgccacctttctggccgacgatgtgcccagcagattcagcggcagcggaagcggcacacagtacagcctgaagatcaactccctgcagagcgaggacgtggcccggtactactgccagcactactacagcaccccctacaccttcggctgcggcaccaagctggaaatcaaaggcgggggaggctccggaggcggcggaagtggaggcggcggaagtggcggaggcggaggggggggaagtgggggcggaggcagtggggggggaggatccgaggtgcagctgctggaatctggcggcggactggtgcagcctggcggatctctgagactgagctgtgccgccagcggcttcaccttcagcacctacgccatgaactgggtgcgccaggcccctggcaaaggcctggaatgggtgtcccggatcagaagcaagtacaacaactacgccacctactacgccgacagcgtgaagggccggttcaccatcagccgggacgacagcaagaacaccctgtacctgcagatgaacagcctgcgggccgaggacaccgccgtgtactattgtgtgcggcacggcaacttcggcaacagctatgtgtcttggtttgcctactggggccagggcaccctcgtgaccgtgtcaagcgctagcgtggccgctccctccgtgttcatcttcccaccttccgacgagcagctgaagtccggcaccgcttctgtcgtgtgcctgctgaacaacttctacccccgcgaggccaaggtgcagtggaaggtggacaacgccctgcagtccggcaacagccaggaatccgtgaccgagcaggactccaaggacagcacctactccctgtcctccaccctgaccctgtccaaggccgactacgagaagcacaaggtgtacgcctgcgaagtgacccaccagggcctgtctagccccgtgaccaagtctttcaaccggggcgagtgctga

SEQ ID NO: 127 - DNA, 699 bp, Chimeric
gaagtgcagctgctggaatccggcggaggactggtgcagcctggcggatctctgagactgtcttgtgccgcctccggcttcaccttctccacctacgccatgaactgggtgcgacaggctcctggcaagggcctggaatgggtgtcccggatcagatccaagtacaacaactacgccacctactacgccgactccgtgaagggccggttcaccatctctcgggacgactccaagaacaccctgtacctgcagatgaactccctgcgggccgaggacaccgccgtgtactattgtgtgcggcacggcaacttcggcaactcctatgtgtcttggtttgcctactggggccagggcaccctcgtgaccgtgtcatctgctagcgtggccgctccctccgtgttcatcttcccaccttccgacgagcagctgaagtccggcaccgcttctgtcgtgtgcctgctgaacaacttctacccccgcgaggccaaggtgcagtggaaggtggacaacgccctgcagtccggcaacagccaggaatccgtgaccgagcaggactccaaggacagcacctactccctgtcctccaccctgaccctgtccaaggccgactacgagaagcacaaggtgtacgcctgcgaagtgacccaccagggcctgtctagccccgtgaccaagtctttcaaccggggcgagtgctga

SEQ ID NO: 128 - DNA, 2871 bp, Chimeric
caagtgcagctgaaagagtccggccctggactggtggcccctagccagagcctgagcatcacctgtaccgtgtccggcttcagcctgaccagctacggcgtgtcatgggtgcgccagcctccaggcaagtgtctggaatggctgggcatcatctggggcgacggcagcaccaattaccacagcgccctgatcagcagactgagcatctccaaggacaacagcaagagccaggtgttcctgaagctgaacagcctgcagaccgacgacaccgccacctactactgcgccaagggcatcaccaccgtggtggacgactactacgctatggactactggggccagggcaccagcgtgacagtgtctagcggaggcggaggatctggcggcggaggaagtggcggagggggatctgggggaggcggaagcgatatccagatgacccagagccctgccagcctgtctgcctctgtgggcgagacagtgaccatcacatgccgggccagcgagaacatcgacagctacctggcctggtatcagcagaagcagggcaagagcccccagctgctggtgtacgccgccacctttctggccgacgatgtgcccagcagattcagcggcagcggaagcggcacacagtacagcctgaagatcaactccctgcagagcgaggacgtggcccggtactactgccagcactactacagcaccccctacaccttcggctgcggcaccaagctggaaatcaaaggaggcggcggaagtgtgcacatgcccctgggcttcctgggccccagacaggccagagtcgtgaacggggggggcggaggcagtggggggggaggatcccaggccgtcgtgacccaggaacccagcctgacagtgtctcctggcggcaccgtgaccctgacatgtggcagttctacaggcgccgtgaccaccagcaactacgccaactgggtgcaggaaaagcccggccaggccttcagaggactgatcggcggcaccaacaagagagcccctggcacccctgccagattcagcggatctctgctgggaggaaaggccgccctgacactgtctggcgcccagccagaagatgaggccgagtactactgcgccctgtggtacagcaacctgtgggtgttcggcggaggcaccaagctgacagtgctgagcagcgcttccaccaagggacccagtgtgttccccctggcccccagctccaagtctacatccggtggcacagctgccctgggatgtctcgtgaaggactactttcctgagcctgtgacagtgtcttggaacagcggagccctgaccagcggagtgcacacattccctgcagtgctgcagagcagcggcctgtatagcctgagcagcgtcgtgaccgtgccttcctctagcctgggaacacagacatatatctgtaatgtgaatcataagcccagtaataccaaagtggataagaaagtggaacctaagagctgcgatggcggaggagggtccggaggcggagggtcccaggtgcagctggtgcagtctggcgccgaagtgaagaaaccaggcgccagcgtgaaggtgtcctgcaaggccagcggctacagcttcaccggctacaccatgaactgggtgcgccaggctcctggacagggcctggaatggatgggcctgatcaccccctacaacggcgccagcagctacaaccagaagttccggggcaaggccaccatgaccgtggacaccagcacctccaccgtgtatatggaactgagcagcctgcggagcgaggacaccgccgtgtactattgtgccagaggcggctacgacggcagaggcttcgattattggggccagggcaccctcgtgaccgtgtcctctgctagcaccaagggcccctccgtgttccccctggcccccagcagcaagagcaccagcggcggcacagccgctctgggctgcctggtcgaggactacttccccgagcccgtgaccgtgtcctggaacagcggagccctgacctccggcgtgcacaccttccccgccgtgctgcagagttctggcctgtatagcctgagcagcgtggtcaccgtgccttctagcagcctgggcacccagacctacatctgcaacgtgaaccacaagcccagcaacaccaaggtggacgagaaggtggagcccaagagctgcgacaaaactcacacatgcccaccgtgcccagcacctgaagctgcagggggaccgtcagtcttcctcttccccccaaaacccaaggacaccctcatgatctcccggacccctgaggtcacatgcgtggtggtggacgtgagccacgaagaccctgaggtcaagttcaactggtacgtggacggcgtggaggtgcataatgccaagacaaagccgcgggaggagcagtacaacagcacgtaccgtgtggtcagcgtcctcaccgtcctgcaccaggactggctgaatggcaaggagtacaagtgcaaggtctccaacaaagccctcggcgcccccatcgagaaaaccatctccaaagccaaagggcagccccgagaaccacaggtgtacaccctgcccccatgccgggatgagctgaccaagaaccaggtcagcctgtggtgcctggtcaaaggcttctatcccagcgacatcgccgtggagtgggagagcaatgggcagccggagaacaactacaagaccacgcctcccgtgctggactccgacggctccttcttcctctacagcaagctcaccgtggacaagagcaggtggcagcaggggaacgtcttctcatgctccgtgatgcatgaggctctgcacaaccactacacgcagaagagcctctccctgtctccgggtaaatga

SEQ ID NO: 129 - DNA, 2871 bp, Chimeric
caagtgcagctgaaagagtccggccctggactggtggcccctagccagagcctgagcatcacctgtaccgtgtccggcttcagcctgaccagctacggcgtgtcatgggtgcgccagcctccaggcaagtgtctggaatggctgggcatcatctggggcgacggcagcaccaattaccacagcgccctgatcagcagactgagcatctccaaggacaacagcaagagccaggtgttcctgaagctgaacagcctgcagaccgacgacaccgccacctactactgcgccaagggcatcaccaccgtggtggacgactactacgctatggactactggggccagggcaccagcgtgacagtgtctagcggaggcggaggatctggcggcggaggaagtggcggagggggatctgggggaggcggaagcgatatccagatgacccagagccctgccagcctgtctgcctctgtgggcgagacagtgaccatcacatgccgggccagcgagaacatcgacagctacctggcctggtatcagcagaagcagggcaagagcccccagctgctggtgtacgccgccacctttctggccgacgatgtgcccagcagattcagcggcagcggaagcggcacacagtacagcctgaagatcaactccctgcagagcgaggacgtggcccggtactactgccagcactactacagcaccccctacaccttcggctgcggcaccaagctggaaatcaaaggcgggggaggctccggaggcggcggaagtggaggcggcggaagtggcggaggcggaggggggggaagtgggggcggaggcagtggggggggaggatcccaggccgtcgtgacccaggaacccagcctgacagtgtctcctggcggcaccgtgaccctgacatgtggcagttctacaggcgccgtgaccaccagcaactacgccaactgggtgcaggaaaagcccggccaggccttcagaggactgatcggcggcaccaacaagagagcccctggcacccctgccagattcagcggatctctgctgggaggaaaggccgccctgacactgtctggcgcccagccagaagatgaggccgagtactactgcgccctgtggtacagcaacctgtgggtgttcggcggaggcaccaagctgacagtgctgagcagcgcttccaccaagggacccagtgtgttccccctggcccccagctccaagtctacatccggtggcacagctgccctgggatgtctcgtgaaggactactttcctgagcctgtgacagtgtcttggaacagcggagccctgaccagcggagtgcacacattccctgcagtgctgcagagcagcggcctgtatagcctgagcagcgtcgtgaccgtgccttcctctagcctgggaacacagacatatatctgtaatgtgaatcataagcccagtaataccaaagtggataagaaagtggaacctaagagctgcgatggcggaggagggtccggaggcggagggtcccaggtgcagctggtgcagtctggcgccgaagtgaagaaaccaggcgccagcgtgaaggtgtcctgcaaggccagcggctacagcttcaccggctacaccatgaactgggtgcgccaggctcctggacagggcctggaatggatgggcctgatcaccccctacaacggcgccagcagctacaaccagaagttccggggcaaggccaccatgaccgtggacaccagcacctccaccgtgtatatggaactgagcagcctgcggagcgaggacaccgccgtgtactattgtgccagaggcggctacgacggcagaggcttcgattattggggccagggcaccctcgtgaccgtgtcctctgctagcaccaagggcccctccgtgttccccctggcccccagcagcaagagcaccagcggcggcacagccgctctgggctgcctggtcgaggactacttccccgagcccgtgaccgtgtcctggaacagcggagccctgacctccggcgtgcacaccttccccgccgtgctgcagagttctggcctgtatagcctgagcagcgtggtcaccgtgccttctagcagcctgggcacccagacctacatctgcaacgtgaaccacaagcccagcaacaccaaggtggacgagaaggtggagcccaagagctgcgacaaaactcacacatgcccaccgtgcccagcacctgaagctgcagggggaccgtcagtcttcctcttccccccaaaacccaaggacaccctcatgatctcccggacccctgaggtcacatgcgtggtggtggacgtgagccacgaagaccctgaggtcaagttcaactggtacgtggacggcgtggaggtgcataatgccaagacaaagccgcgggaggagcagtacaacagcacgtaccgtgtggtcagcgtcctcaccgtcctgcaccaggactggctgaatggcaaggagtacaagtgcaaggtctccaacaaagccctcggcgcccccatcgagaaaaccatctccaaagccaaagggcagccccgagaaccacaggtgtacaccctgcccccatgccgggatgagctgaccaagaaccaggtcagcctgtggtgcctggtcaaaggcttctatcccagcgacatcgccgtggagtgggagagcaatgggcagccggagaacaactacaagaccacgcctcccgtgctggactccgacggctccttcttcctctacagcaagctcaccgtggacaagagcaggtggcagcaggggaacgtcttctcatgctccgtgatgcatgaggctctgcacaaccactacacgcagaagagcctctccctgtctccgggtaaatga

SEQ ID NO: 130 - DNA, 2025 bp, Chimeric
caggccgtcgtgacccaggaacccagcctgacagtgtctcctggcggcaccgtgaccctgacatgtggcagttctacaggcgccgtgaccaccagcaactacgccaactgggtgcaggaaaagcccggccaggccttcagaggactgatcggcggcaccaacaagagagcccctggcacccctgccagattctccggttctctgctgggcggcaaggctgccctgactctgtctggtgctcagcctgaggacgaggccgagtactactgcgccctgtggtactccaacctgtgggtgttcggcggaggcaccaagctgaccgtgctgtccagcgcttccaccaagggacccagtgtgttccccctggcccccagctccaagtctacatccggtggcacagctgccctgggatgtctcgtgaaggactactttcctgagcctgtgacagtgtcttggaacagcggagccctgaccagcggagtgcacacattccctgcagtgctgcagagcagcggcctgtatagcctgagcagcgtcgtgaccgtgccttcctctagcctgggaacacagacatatatctgtaatgtgaatcataagcccagtaataccaaagtggataagaaagtggaacctaagagctgcgatggcggaggagggtccggaggcggagggtcccaggtgcagctggtgcagtctggcgccgaagtgaagaaaccaggcgccagcgtgaaggtgtcctgcaaggccagcggctacagcttcaccggctacaccatgaactgggtgcgccaggctcctggacagggcctggaatggatgggcctgatcaccccctacaacggcgccagcagctacaaccagaagttccggggcaaggccaccatgaccgtggacaccagcacctccaccgtgtatatggaactgagcagcctgcggagcgaggacaccgccgtgtactattgtgccagaggcggctacgacggcagaggcttcgattattggggccagggcaccctcgtgaccgtgtcctctgctagcaccaagggcccctccgtgttccccctggcccccagcagcaagagcaccagcggcggcacagccgctctgggctgcctggtcgaggactacttccccgagcccgtgaccgtgtcctggaacagcggagccctgacctccggcgtgcacaccttccccgccgtgctgcagagttctggcctgtatagcctgagcagcgtggtcaccgtgccttctagcagcctgggcacccagacctacatctgcaacgtgaaccacaagcccagcaacaccaaggtggacgagaaggtggagcccaagagctgcgacaaaactcacacatgcccaccgtgcccagcacctgaagctgcagggggaccgtcagtcttcctcttccccccaaaacccaaggacaccctcatgatctcccggacccctgaggtcacatgcgtggtggtggacgtgagccacgaagaccctgaggtcaagttcaactggtacgtggacggcgtggaggtgcataatgccaagacaaagccgcgggaggagcagtacaacagcacgtaccgtgtggtcagcgtcctcaccgtcctgcaccaggactggctgaatggcaaggagtacaagtgcaaggtctccaacaaagccctcggcgcccccatcgagaaaaccatctccaaagccaaagggcagccccgagaaccacaggtgtacaccctgcccccatgccgggatgagctgaccaagaaccaggtcagcctgtggtgcctggtcaaaggcttctatcccagcgacatcgccgtggagtgggagagcaatgggcagccggagaacaactacaagaccacgcctcccgtgctggactccgacggctccttcttcctctacagcaagctcaccgtggacaagagcaggtggcagcaggggaacgtcttctcatgctccgtgatgcatgaggctctgcacaaccactacacgcagaagagcctctccctgtctccgggtaaatga

SEQ ID NO: 131 - DNA, 2916 bp, Chimeric
caagtgcagctgaaagagtccggccctggactggtggcccctagccagagcctgagcatcacctgtaccgtgtccggcttcagcctgaccagctacggcgtgtcatgggtgcgccagcctccaggcaagtgtctggaatggctgggcatcatctggggcgacggcagcaccaattaccacagcgccctgatcagcagactgagcatctccaaggacaacagcaagagccaggtgttcctgaagctgaacagcctgcagaccgacgacaccgccacctactactgcgccaagggcatcaccaccgtggtggacgactactacgctatggactactggggccagggcaccagcgtgacagtgtctagcggaggcggaggatctggcggcggaggaagtggcggagggggatctgggggaggcggaagcgatatccagatgacccagagccctgccagcctgtctgcctctgtgggcgagacagtgaccatcacatgccgggccagcgagaacatcgacagctacctggcctggtatcagcagaagcagggcaagagcccccagctgctggtgtacgccgccacctttctggccgacgatgtgcccagcagattcagcggcagcggaagcggcacacagtacagcctgaagatcaactccctgcagagcgaggacgtggcccggtactactgccagcactactacagcaccccctacaccttcggctgcggcaccaagctggaaatcaaaggcgggggaggctccggaggcggcggaagtggaggcggcggaagtttcgtgggggggaccgggggcggaggcagtggggggggaggatccgggggatccgaggtgcagctgctggaatctggcggcggactggtgcagcctggcggatctctgagactgagctgtgccgccagcggcttcaccttcagcacctacgccatgaactgggtgcgccaggcccctggcaaaggcctggaatgggtgtcccggatcagaagcaagtacaacaactacgccacctactacgccgacagcgtgaagggccggttcaccatcagccgggacgacagcaagaacaccctgtacctgcagatgaacagcctgcgggccgaggacaccgccgtgtactattgtgtgcggcacggcaacttcggcaacagctatgtgtcttggtttgcctactggggccagggcaccctcgtgaccgtgtcaagcgctagcacaaagggccctagcgtgttccctctggcccccagcagcaagagcacaagcggcggaacagccgccctgggctgcctcgtgaaggactacttccccgagcccgtgacagtgtcttggaacagcggagccctgacaagcggcgtgcacaccttccctgccgtgctgcagagcagcggcctgtactccctgagcagcgtggtcaccgtgcctagcagcagcctgggcacccagacctacatctgcaacgtgaaccacaagcccagcaacaccaaagtggacaagaaggtggagcccaagagctgtgatggcggaggagggtccgggggcggaggatccgaggtgcaattggttgaatctggtggtggtctggtaaaaccgggcggttccctgcgtctgagctgcgcggcttccgggttcaccttctccaacgcgtggatgagctgggttcgccaggccccgggcaaaggcctcgagtgggttggtcgtatcaagtctaaaactgacggtggcaccacggattacgcggctccagttaaaggtcgttttaccatttcccgcgacgatagcaaaaacactctgtatctgcagatgaactctctgaaaactgaagacaccgcagtctactactgtactaccccgtgggaatggtcttggtacgattattggggccagggcacgctggttacggtgtctagcgctagtaccaagggccccagcgtgttccccctggcacccagcagcaagagcacatctggcggaacagccgctctgggctgtctggtgaaagactacttccccgagcccgtgaccgtgtcttggaactctggcgccctgaccagcggcgtgcacacctttccagccgtgctgcagagcagcggcctgtactccctgtcctccgtggtcaccgtgccctctagctccctgggaacacagacatatatctgtaatgtcaatcacaagccttccaacaccaaagtcgataagaaagtcgagcccaagagctgcgacaaaactcacacatgcccaccgtgcccagcacctgaagctgcagggggaccgtcagtcttcctcttccccccaaaacccaaggacaccctcatgatctcccggacccctgaggtcacatgcgtggtggtggacgtgagccacgaagaccctgaggtcaagttcaactggtacgtggacggcgtggaggtgcataatgccaagacaaagccgcgggaggagcagtacaacagcacgtaccgtgtggtcagcgtcctcaccgtcctgcaccaggactggctgaatggcaaggagtacaagtgcaaggtctccaacaaagccctcggcgcccccatcgagaaaaccatctccaaagccaaagggcagccccgagaaccacaggtgtacaccctgcccccatgccgggatgagctgaccaagaaccaggtcagcctgtggtgcctggtcaaaggcttctatcccagcgacatcgccgtggagtgggagagcaatgggcagccggagaacaactacaagaccacgcctcccgtgctggactccgacggctccttcttcctctacagcaagctcaccgtggacaagagcaggtggcagcaggggaacgtcttctcatgctccgtgatgcatgaggctctgcacaaccactacacgcagaagagcctctccctgtctccgggtaaatga

SEQ ID NO: 132 - protein, 449 aa, Chimeric
EVQLVESGGGLVQPGGSLRLSCAASGFTFNDYTMDWVRQAPGKGLEWVADVNPNSGGSIVNRRFKGRFTLSVDRSKNTLYLQMNSLRAEDTAVYYCARNLGPFFYFDYWGQGTLVTVSSASTKGPSVFPLAPSSKSTSGGTAALGCLVEDYFPEPVTVSWNSGALTSGVHTFPAVLQSSGLYSLSSVVTVPSSSLGTQTYICNVNHKPSNTKVDEKVEPKSCDKTHTCPPCPAPEAAGGPSVFLFPPKPKDTLMISRTPEVTCVVVDVSHEDPEVKFNWYVDGVEVHNAKTKPREEQYNSTYRVVSVLTVLHQDWLNGKEYKCKVSNKALGAPIEKTISKAKGQPREPQVCTLPPSRDELTKNQVSLSCAVKGFYPSDIAVEWESNGQPENNYKTTPPVLDSDGSFFLVSKLTVDKSRWQQGNVFSCSVMHEALHNHYTQKSLSLSPGK

SEQ ID NO: 133 - protein, 214 aa, Chimeric
DIQMTQSPSSLSASVGDRVTITCKASQDVSTAVAWYQQKPGKAPKLLIYSASFRYTGVPSRFSGSRSGTDFTLTISSLQPEDFATYYCQQHYTTPPTFGQGTKVEIKRTVAAPSVFIFPPSDRKLKSGTASVVCLLNNFYPREAKVQWKVDNALQSGNSQESVTEQDSKDSTYSLSSTLTLSKADYEKHKVYACEVTHQGLSSPVTKSFNRGEC

SEQ ID NO: 134 - protein, 675 aa, Chimeric
QAVVTQEPSLTVSPGGTVTLTCGSSTGAVTTSNYANWVQEKPGQAFRGLIGGTNKRAPGTPARFSGSLLGGKAALTLSGAQPEDEAEYYCALWYSNLWVFGGGTKLTVLSSASTKGPSVFPLAPSSKSTSGGTAALGCLVKDYFPEPVTVSWNSGALTSGVHTFPAVLQSSGLYSLSSVVTVPSSSLGTQTYICNVNHKPSNTKVDKKVEPKSCDGGGGSGGGGSEVQLVESGGGLVQPGGSLRLSCAASGFNIKDTYIHWVRQAPGKGLEWVARIYPTNGYTRYADSVKGRFTISADTSKNTAYLQMNSLRAEDTAVYYCSRWGGEGFYAMDYWGQGTLVTVSSASTKGPSVFPLAPSSKSTSGGTAALGCLVEDYFPEPVTVSWNSGALTSGVHTFPAVLQSSGLYSLSSVVTVPSSSLGTQTYICNVNHKPSNTKVDEKVEPKSCDKTHTCPPCPAPEAAGGPSVFLFPPKPKDTLMISRTPEVTCVVVDVSHEDPEVKFNWYVDGVEVHNAKTKPREEQYNSTYRVVSVLTVLHQDWLNGKEYKCKVSNKALGAPIEKTISKAKGQPREPQVYTLPPCRDELTKNQVSLWCLVKGFYPSDIAVEWESNGQPENNYKTTPPVLDSDGSFFLYSKLTVDKSRWQQGNVFSCSVMHEALHNHYTQKSLSLSPGK

SEQ ID NO: 135 - protein, 957 aa, Chimeric
QVQLKESGPGLVAPSQSLSITCTVSGFSLTSYGVSWVRQPPGKCLEWLGIIWGDGSTNYHSALISRLSISKDNSKSQVFLKLNSLQTDDTATYYCAKGITTVVDDYYAMDYWGQGTSVTVSSGGGGSGGGGSGGGGSGGGGSDIQMTQSPASLSASVGETVTITCRASENIDSYLAWYQQKQGKSPQLLVYAATFLADDVPSRFSGSGSGTQYSLKINSLQSEDVARYYCQHYYSTPYTFGCGTKLEIKGGGGSGGGGSGGGGSGGGGGGGSGGGGSGGGGSQAVVTQEPSLTVSPGGTVTLTCGSSTGAVTTSNYANWVQEKPGQAFRGLIGGTNKRAPGTPARFSGSLLGGKAALTLSGAQPEDEAEYYCALWYSNLWVFGGGTKLTVLSSASTKGPSVFPLAPSSKSTSGGTAALGCLVKDYFPEPVTVSWNSGALTSGVHTFPAVLQSSGLYSLSSVVTVPSSSLGTQTYICNVNHKPSNTKVDKKVEPKSCDGGGGSGGGGSEVQLVESGGGLVQPGGSLRLSCAASGFNIKDTYIHWVRQAPGKGLEWVARIYPTNGYTRYADSVKGRFTISADTSKNTAYLQMNSLRAEDTAVYYCSRWGGEGFYAMDYWGQGTLVTVSSASTKGPSVFPLAPSSKSTSGGTAALGCLVEDYFPEPVTVSWNSGALTSGVHTFPAVLQSSGLYSLSSVVTVPSSSLGTQTYICNVNHKPSNTKVDEKVEPKSCDKTHTCPPCPAPEAAGGPSVFLFPPKPKDTLMISRTPEVTCVVVDVSHEDPEVKFNWYVDGVEVHNAKTKPREEQYNSTYRVVSVLTVLHQDWLNGKEYKCKVSNKALGAPIEKTISKAKGQPREPQVYTLPPCRDELTKNQVSLWCLVKGFYPSDIAVEWESNGQPENNYKTTPPVLDSDGSFFLYSKLTVDKSRWQQGNVFSCSVMHEALHNHYTQKSLSLSPGK

SEQ ID NO: 136 - protein, 957 aa, Chimeric
QVQLKESGPGLVAPSQSLSITCTVSGFSLTSYGVSWVRQPPGKCLEWLGIIWGDGSTNYHSALISRLSISKDNSKSQVFLKLNSLQTDDTATYYCAKGITTVVDDYYAMDYWGQGTSVTVSSGGGGSGGGGSGGGGSGGGGSDIQMTQSPASLSASVGETVTITCRASENIDSYLAWYQQKQGKSPQLLVYAATFLADDVPSRFSGSGSGTQYSLKINSLQSEDVARYYCQHYYSTPYTFGCGTKLEIKGGGGSVHMPLGFLGPRQARVVNGGGGGSGGGGSQAVVTQEPSLTVSPGGTVTLTCGSSTGAVTTSNYANWVQEKPGQAFRGLIGGTNKRAPGTPARFSGSLLGGKAALTLSGAQPEDEAEYYCALWYSNLWVFGGGTKLTVLSSASTKGPSVFPLAPSSKSTSGGTAALGCLVKDYFPEPVTVSWNSGALTSGVHTFPAVLQSSGLYSLSSVVTVPSSSLGTQTYICNVNHKPSNTKVDKKVEPKSCDGGGGSGGGGSEVQLVESGGGLVQPGGSLRLSCAASGFNIKDTYIHWVRQAPGKGLEWVARIYPTNGYTRYADSVKGRFTISADTSKNTAYLQMNSLRAEDTAVYYCSRWGGEGFYAMDYWGQGTLVTVSSASTKGPSVFPLAPSSKSTSGGTAALGCLVEDYFPEPVTVSWNSGALTSGVHTFPAVLQSSGLYSLSSVVTVPSSSLGTQTYICNVNHKPSNTKVDEKVEPKSCDKTHTCPPCPAPEAAGGPSVFLFPPKPKDTLMISRTPEVTCVVVDVSHEDPEVKFNWYVDGVEVHNAKTKPREEQYNSTYRVVSVLTVLHQDWLNGKEYKCKVSNKALGAPIEKTISKAKGQPREPQVYTLPPCRDELTKNQVSLWCLVKGFYPSDIAVEWESNGQPENNYKTTPPVLDSDGSFFLYSKLTVDKSRWQQGNVFSCSVMHEALHNHYTQKSLSLSPGK

SEQ ID NO: 137 - protein, 449 aa, Chimeric
QVQLVQSGAEVKKPGASVKVSCKASGYTFTSYYMHWVRQAPGQGLEWMGIINPSGGSTSYAQKFQGRVTMTHDTSTSTVYMELSSLRSEDTAVYYCARSFFTGFHLDYWGQGTLVTVSSASTKGPSVFPLAPSSKSTSGGTAALGCLVEDYFPEPVTVSWNSGALTSGVHTFPAVLQSSGLYSLSSVVTVPSSSLGTQTYICNVNHKPSNTKVDEKVEPKSCDKTHTCPPCPAPEAAGGPSVFLFPPKPKDTLMISRTPEVTCVVVDVSHEDPEVKFNWYVDGVEVHNAKTKPREEQYNSTYRVVSVLTVLHQDWLNGKEYKCKVSNKALGAPIEKTISKAKGQPREPQVCTLPPSRDELTKNQVSLSCAVKGFYPSDIAVEWESNGQPENNYKTTPPVLDSDGSFFLVSKLTVDKSRWQQGNVFSCSVMHEALHNHYTQKSLSLSPGK

SEQ ID NO: 138 - protein, 216 aa, Chimeric
EIVLTQSPGTLSLSPGERATLSCRASQSVSSSYLAWYQQKPGQAPRLLIYGASSRATGIPDRFSGSGSGTDFTLTISRLEPEDFAVYYCQQYTNEHYYTFGQGTKVEIKRTVAAPSVFIFPPSDRKLKSGTASVVCLLNNFYPREAKVQWKVDNALQSGNSQESVTEQDSKDSTYSLSSTLTLSKADYEKHKVYACEVTHQGLSSPVTKSFNRGEC

SEQ ID NO: 139 - protein, 956 aa, Chimeric
QVQLKESGPGLVAPSQSLSITCTVSGFSLTSYGVSWVRQPPGKCLEWLGIIWGDGSTNYHSALISRLSISKDNSKSQVFLKLNSLQTDDTATYYCAKGITTVVDDYYAMDYWGQGTSVTVSSGGGGSGGGGSGGGGSGGGGSDIQMTQSPASLSASVGETVTITCRASENIDSYLAWYQQKQGKSPQLLVYAATFLADDVPSRFSGSGSGTQYSLKINSLQSEDVARYYCQHYYSTPYTFGCGTKLEIKGGGGSVHMPLGFLGPRQARVVNGGGGGSGGGGSQAVVTQEPSLTVSPGGTVTLTCGSSTGAVTTSNYANWVQEKPGQAFRGLIGGTNKRAPGTPARFSGSLLGGKAALTLSGAQPEDEAEYYCALWYSNLWVFGGGTKLTVLSSASTKGPSVFPLAPSSKSTSGGTAALGCLVKDYFPEPVTVSWNSGALTSGVHTFPAVLQSSGLYSLSSVVTVPSSSLGTQTYICNVNHKPSNTKVDKKVEPKSCDGGGGSGGGGSQVQLVQSGAEVKKPGASVKVSCKASGYTFTSYYMHWVRQAPGQGLEWMGIINPSGGSTSYAQKFQGRVTMTHDTSTSTVYMELSSLRSEDTAVYYCARSFFTGFHLDYWGQGTLVTVSSASTKGPSVFPLAPSSKSTSGGTAALGCLVEDYFPEPVTVSWNSGALTSGVHTFPAVLQSSGLYSLSSVVTVPSSSLGTQTYICNVNHKPSNTKVDEKVEPKSCDKTHTCPPCPAPEAAGGPSVFLFPPKPKDTLMISRTPEVTCVVVDVSHEDPEVKFNWYVDGVEVHNAKTKPREEQYNSTYRVVSVLTVLHQDWLNGKEYKCKVSNKALGAPIEKTISKAKGQPREPQVYTLPPCRDELTKNQVSLWCLVKGFYPSDIAVEWESNGQPENNYKTTPPVLDSDGSFFLYSKLTVDKSRWQQGNVFSCSVMHEALHNHYTQKSLSLSPGK

SEQ ID NO: 140 - protein, 956 aa, Chimeric
QVQLKESGPGLVAPSQSLSITCTVSGFSLTSYGVSWVRQPPGKCLEWLGIIWGDGSTNYHSALISRLSISKDNSKSQVFLKLNSLQTDDTATYYCAKGITTVVDDYYAMDYWGQGTSVTVSSGGGGSGGGGSGGGGSGGGGSDIQMTQSPASLSASVGETVTITCRASENIDSYLAWYQQKQGKSPQLLVYAATFLADDVPSRFSGSGSGTQYSLKINSLQSEDVARYYCQHYYSTPYTFGCGTKLEIKGGGGSGGGGSGGGGSGGGGGGGSGGGGSGGGGSQAVVTQEPSLTVSPGGTVTLTCGSSTGAVTTSNYANWVQEKPGQAFRGLIGGTNKRAPGTPARFSGSLLGGKAALTLSGAQPEDEAEYYCALWYSNLWVFGGGTKLTVLSSASTKGPSVFPLAPSSKSTSGGTAALGCLVKDYFPEPVTVSWNSGALTSGVHTFPAVLQSSGLYSLSSVVTVPSSSLGTQTYICNVNHKPSNTKVDKKVEPKSCDGGGGSGGGGSQVQLVQSGAEVKKPGASVKVSCKASGYTFTSYYMHWVRQAPGQGLEWMGIINPSGGSTSYAQKFQGRVTMTHDTSTSTVYMELSSLRSEDTAVYYCARSFFTGFHLDYWGQGTLVTVSSASTKGPSVFPLAPSSKSTSGGTAALGCLVEDYFPEPVTVSWNSGALTSGVHTFPAVLQSSGLYSLSSVVTVPSSSLGTQTYICNVNHKPSNTKVDEKVEPKSCDKTHTCPPCPAPEAAGGPSVFLFPPKPKDTLMISRTPEVTCVVVDVSHEDPEVKFNWYVDGVEVHNAKTKPREEQYNSTYRVVSVLTVLHQDWLNGKEYKCKVSNKALGAPIEKTISKAKGQPREPQVYTLPPCRDELTKNQVSLWCLVKGFYPSDIAVEWESNGQPENNYKTTPPVLDSDGSFFLYSKLTVDKSRWQQGNVFSCSVMHEALHNHYTQKSLSLSPGK

SEQ ID NO: 141 - protein, 674 aa, Chimeric
QAVVTQEPSLTVSPGGTVTLTCGSSTGAVTTSNYANWVQEKPGQAFRGLIGGTNKRAPGTPARFSGSLLGGKAALTLSGAQPEDEAEYYCALWYSNLWVFGGGTKLTVLSSASTKGPSVFPLAPSSKSTSGGTAALGCLVKDYFPEPVTVSWNSGALTSGVHTFPAVLQSSGLYSLSSVVTVPSSSLGTQTYICNVNHKPSNTKVDKKVEPKSCDGGGGSGGGGSQVQLVQSGAEVKKPGASVKVSCKASGYTFTSYYMHWVRQAPGQGLEWMGIINPSGGSTSYAQKFQGRVTMTHDTSTSTVYMELSSLRSEDTAVYYCARSFFTGFHLDYWGQGTLVTVSSASTKGPSVFPLAPSSKSTSGGTAALGCLVEDYFPEPVTVSWNSGALTSGVHTFPAVLQSSGLYSLSSVVTVPSSSLGTQTYICNVNHKPSNTKVDEKVEPKSCDKTHTCPPCPAPEAAGGPSVFLFPPKPKDTLMISRTPEVTCVVVDVSHEDPEVKFNWYVDGVEVHNAKTKPREEQYNSTYRVVSVLTVLHQDWLNGKEYKCKVSNKALGAPIEKTISKAKGQPREPQVYTLPPCRDELTKNQVSLWCLVKGFYPSDIAVEWESNGQPENNYKTTPPVLDSDGSFFLYSKLTVDKSRWQQGNVFSCSVMHEALHNHYTQKSLSLSPGK

SEQ ID NO: 142 - protein, 5 aa, Chimeric
DYTMD

SEQ ID NO: 143 - protein, 17 aa, Chimeric
DVNPNSGGSIVNRRFKG

SEQ ID NO: 144 - protein, 10 aa, Chimeric
NLGPFFYFDY

SEQ ID NO: 145 - protein, 7 aa, Chimeric
TSNYANW

SEQ ID NO: 146 - protein, 20 aa, Chimeric
GTNKRAPGTPARFSGSLLGG

SEQ ID NO: 147 - protein, 5 aa, Chimeric
TKLTV

SEQ ID NO: 148 - protein, 11 aa, Chimeric
KASQDVSTAVA

SEQ ID NO: 149 - protein, 7 aa, Chimeric
SASFRYT

SEQ ID NO: 150 - protein, 9 aa, Chimeric
QQHYTTPPT

SEQ ID NO: 151 - protein, 5 aa, Chimeric
SYYMH

SEQ ID NO: 152 - protein, 17 aa, Chimeric
IINPSGGSTSYAQKFQG

SEQ ID NO: 153 - protein, 10 aa, Chimeric
SFFTGFHLDY

SEQ ID NO: 154 - protein, 12 aa, Chimeric
RASQSVSSSYLA

SEQ ID NO: 155 - protein, 7 aa, Chimeric
GASSRAT

SEQ ID NO: 156 - protein, 10 aa, Chimeric
QQYTNEHYYT

SEQ ID NO: 157 - protein, 119 aa, Chimeric
QVQLVQSGAEVKKPGASVKVSCKASGYTFTSYYMHWVRQAPGQGLEWMGIINPSGGSTSYAQKFQGRVTMTHDTSTSTVYMELSSLRSEDTAVYYCARSFFTGFHLDYWGQGTLVTVSS

SEQ ID NO: 158 - protein, 109 aa, Chimeric
EIVLTQSPGTLSLSPGERATLSCRASQSVSSSYLAWYQQKPGQAPRLLIYGASSRATGIPDRFSGSGSGTDFTLTISRLEPEDFAVYYCQQYTNEHYYTFGQGTKVEIK

SEQ ID NO: 159 - protein, 119 aa, Chimeric
EVQLVESGGGLVQPGGSLRLSCAASGFTFNDYTMDWVRQAPGKGLEWVADVNPNSGGSIVNRRFKGRFTLSVDRSKNTLYLQMNSLRAEDTAVYYCARNLGPFFYFDYWGQGTLVTVSS

SEQ ID NO: 160 - protein, 120 aa, Chimeric
EVQLVESGGGLVQPGGSLRLSCAASGFNIKDTYIHWVRQAPGKGLEWVARIYPTNGYTRYADSVKGRFTISADTSKNTAYLQMNSLRAEDTAVYYCSRWGGEGFYAMDYWGQGTLVTVSS

SEQ ID NO: 161 - protein, 107 aa, Chimeric
DIQMTQSPSSLSASVGDRVTITCKASQDVSTAVAWYQQKPGKAPKLLIYSASFRYTGVPSRFSGSRSGTDFTLTISSLQPEDFATYYCQQHYTTPPTFGQGTKVEIK

SEQ ID NO: 162 - DNA, 1350 bp, Chimeric
gaagttcagctggttgaaagcggtggtggtctggttcagcctggtggtagcctgcgtctgagctgtgcagcaagcggttttacctttaacgattataccatggattgggttcgtcaggcaccgggtaaaggtctggaatgggttgcagatgttaatccgaatagcggtggtagcattgttaaccgtcgttttaaaggtcgttttaccctgagcgttgatcgtagcaaaaataccctgtatctgcaaatgaatagtctgcgtgcagaggataccgcagtgtattattgtgcacgtaacctgggtccgttcttctactttgattattggggtcagggcaccctggttaccgttagcagcgctagcaccaagggcccctccgtgttccccctggcccccagcagcaagagcaccagcggcggcacagccgctctgggctgcctggtcgaggactacttccccgagcccgtgaccgtgtcctggaacagcggagccctgacctccggcgtgcacaccttccccgccgtgctgcagagttctggcctgtatagcctgagcagcgtggtcaccgtgccttctagcagcctgggcacccagacctacatctgcaacgtgaaccacaagcccagcaacaccaaggtggacgagaaggtggagcccaagagctgcgacaaaactcacacatgcccaccgtgcccagcacctgaagctgcagggggaccgtcagtcttcctcttccccccaaaacccaaggacaccctcatgatctcccggacccctgaggtcacatgcgtggtggtggacgtgagccacgaagaccctgaggtcaagttcaactggtacgtggacggcgtggaggtgcataatgccaagacaaagccgcgggaggagcagtacaacagcacgtaccgtgtggtcagcgtcctcaccgtcctgcaccaggactggctgaatggcaaggagtacaagtgcaaggtctccaacaaagccctcggcgcccccatcgagaaaaccatctccaaagccaaagggcagccccgagaaccacaggtgtgcaccctgcccccatcccgggatgagctgaccaagaaccaggtcagcctctcgtgcgcagtcaaaggcttctatcccagcgacatcgccgtggagtgggagagcaatgggcagccggagaacaactacaagaccacgcctcccgtgctggactccgacggctccttcttcctcgtgagcaagctcaccgtggacaagagcaggtggcagcaggggaacgtcttctcatgctccgtgatgcatgaggctctgcacaaccactacacgcagaagagcctctccctgtctccgggtaaatga

SEQ ID NO: 163 - DNA, 645 bp, Chimeric
gacatccagatgacccagagccccagcagcctgtctgccagcgtgggcgacagagtgaccatcacatgcaaggccagccaggacgtgtccacagccgtggcctggtatcagcagaagcctggcaaggcccccaagctgctgatctacagcgccagcttccggtacaccggcgtgcccagcagattcagcggcagcagatccggcaccgacttcaccctgaccatcagctccctgcagcccgaggacttcgccacctactactgccagcagcactacaccaccccccccacatttggccagggcaccaaggtggaaatcaagcgtacggtggctgcaccatctgtcttcatcttcccgccatctgatcggaagttgaaatctggaactgcctctgttgtgtgcctgctgaataacttctatcccagagaggccaaagtacagtggaaggtggataacgccctccaatcgggtaactcccaggagagtgtcacagagcaggacagcaaggacagcacctacagcctcagcagcaccctgacgctgagcaaagcagactacgagaaacacaaagtctacgcctgcgaagtcacccatcagggcctgagctcgcccgtcacaaagagcttcaacaggggagagtgttag

SEQ ID NO: 164 - DNA, 2874 bp, Chimeric
caagtgcagctgaaagagtccggccctggactggtggcccctagccagagcctgagcatcacctgtaccgtgtccggcttcagcctgaccagctacggcgtgtcatgggtgcgccagcctccaggcaagtgtctggaatggctgggcatcatctggggcgacggcagcaccaattaccacagcgccctgatcagcagactgagcatctccaaggacaacagcaagagccaggtgttcctgaagctgaacagcctgcagaccgacgacaccgccacctactactgcgccaagggcatcaccaccgtggtggacgactactacgctatggactactggggccagggcaccagcgtgacagtgtctagcggaggcggaggatctggcggcggaggaagtggcggagggggatctgggggaggcggaagcgatatccagatgacccagagccctgccagcctgtctgcctctgtgggcgagacagtgaccatcacatgccgggccagcgagaacatcgacagctacctggcctggtatcagcagaagcagggcaagagcccccagctgctggtgtacgccgccacctttctggccgacgatgtgcccagcagattcagcggcagcggaagcggcacacagtacagcctgaagatcaactccctgcagagcgaggacgtggcccggtactactgccagcactactacagcaccccctacaccttcggctgcggcaccaagctggaaatcaaaggcgggggaggctccggaggcggcggaagtggaggcggcggaagtggcggaggcggaggggggggaagtgggggcggaggcagtggggggggaggatcccaggccgtcgtgacccaggaacccagcctgacagtgtctcctggcggcaccgtgaccctgacatgtggcagttctacaggcgccgtgaccaccagcaactacgccaactgggtgcaggaaaagcccggccaggccttcagaggactgatcggcggcaccaacaagagagcccctggcacccctgccagattcagcggatctctgctgggaggaaaggccgccctgacactgtctggcgcccagccagaagatgaggccgagtactactgcgccctgtggtacagcaacctgtgggtgttcggcggaggcaccaagctgacagtgctgagcagcgcttccaccaagggacccagtgtgttccccctggcccccagctccaagtctacatccggtggcacagctgccctgggatgtctcgtgaaggactactttcctgagcctgtgacagtgtcttggaacagcggagccctgaccagcggagtgcacacattccctgcagtgctgcagagcagcggcctgtatagcctgagcagcgtcgtgaccgtgccttcctctagcctgggaacacagacatatatctgtaatgtgaatcataagcccagtaataccaaagtggataagaaagtggaacctaagagctgcgatggcggaggagggtccggaggcggagggtccgaggtccagctggtcgagtctggaggaggactggtgcagccaggcggatctctgagactgagctgcgccgccagcggattcaacatcaaggacacctacatccactgggtgaggcaggcccctggaaagggactggagtgggtggccagaatctaccccaccaacggctacacaagatacgccgacagcgtgaagggcagattcaccatcagcgccgacaccagcaagaacaccgcctacctgcagatgaacagcctgagagccgaggacacagccgtgtactactgctctagatggggaggcgagggcttctacgccatggactactggggacagggcacactggtgaccgtgtccagcgctagcaccaagggcccctccgtgttccccctggcccccagcagcaagagcaccagcggcggcacagccgctctgggctgcctggtcgaggactacttccccgagcccgtgaccgtgtcctggaacagcggagccctgacctccggcgtgcacaccttccccgccgtgctgcagagttctggcctgtatagcctgagcagcgtggtcaccgtgccttctagcagcctgggcacccagacctacatctgcaacgtgaaccacaagcccagcaacaccaaggtggacgagaaggtggagcccaagagctgcgacaaaactcacacatgcccaccgtgcccagcacctgaagctgcagggggaccgtcagtcttcctcttccccccaaaacccaaggacaccctcatgatctcccggacccctgaggtcacatgcgtggtggtggacgtgagccacgaagaccctgaggtcaagttcaactggtacgtggacggcgtggaggtgcataatgccaagacaaagccgcgggaggagcagtacaacagcacgtaccgtgtggtcagcgtcctcaccgtcctgcaccaggactggctgaatggcaaggagtacaagtgcaaggtctccaacaaagccctcggcgcccccatcgagaaaaccatctccaaagccaaagggcagccccgagaaccacaggtgtacaccctgcccccatgccgggatgagctgaccaagaaccaggtcagcctgtggtgcctggtcaaaggcttctatcccagcgacatcgccgtggagtgggagagcaatgggcagccggagaacaactacaagaccacgcctcccgtgctggactccgacggctccttcttcctctacagcaagctcaccgtggacaagagcaggtggcagcaggggaacgtcttctcatgctccgtgatgcatgaggctctgcacaaccactacacgcagaagagcctctccctgtctccgggtaaatga

SEQ ID NO: 165 - DNA, 2874 bp, Chimeric
caagtgcagctgaaagagtccggccctggactggtggcccctagccagagcctgagcatcacctgtaccgtgtccggcttcagcctgaccagctacggcgtgtcatgggtgcgccagcctccaggcaagtgtctggaatggctgggcatcatctggggcgacggcagcaccaattaccacagcgccctgatcagcagactgagcatctccaaggacaacagcaagagccaggtgttcctgaagctgaacagcctgcagaccgacgacaccgccacctactactgcgccaagggcatcaccaccgtggtggacgactactacgctatggactactggggccagggcaccagcgtgacagtgtctagcggaggcggaggatctggcggcggaggaagtggcggagggggatctgggggaggcggaagcgatatccagatgacccagagccctgccagcctgtctgcctctgtgggcgagacagtgaccatcacatgccgggccagcgagaacatcgacagctacctggcctggtatcagcagaagcagggcaagagcccccagctgctggtgtacgccgccacctttctggccgacgatgtgcccagcagattcagcggcagcggaagcggcacacagtacagcctgaagatcaactccctgcagagcgaggacgtggcccggtactactgccagcactactacagcaccccctacaccttcggctgcggcaccaagctggaaatcaaaggaggcggcggaagtgtgcacatgcccctgggcttcctgggccccagacaggccagagtcgtgaacggggggggcggaggcagtggggggggaggatcccaggccgtcgtgacccaggaacccagcctgacagtgtctcctggcggcaccgtgaccctgacatgtggcagttctacaggcgccgtgaccaccagcaactacgccaactgggtgcaggaaaagcccggccaggccttcagaggactgatcggcggcaccaacaagagagcccctggcacccctgccagattcagcggatctctgctgggaggaaaggccgccctgacactgtctggcgcccagccagaagatgaggccgagtactactgcgccctgtggtacagcaacctgtgggtgttcggcggaggcaccaagctgacagtgctgagcagcgcttccaccaagggacccagtgtgttccccctggcccccagctccaagtctacatccggtggcacagctgccctgggatgtctcgtgaaggactactttcctgagcctgtgacagtgtcttggaacagcggagccctgaccagcggagtgcacacattccctgcagtgctgcagagcagcggcctgtatagcctgagcagcgtcgtgaccgtgccttcctctagcctgggaacacagacatatatctgtaatgtgaatcataagcccagtaataccaaagtggataagaaagtggaacctaagagctgcgatggcggaggagggtccggaggcggagggtccgaggtccagctggtcgagtctggaggaggactggtgcagccaggcggatctctgagactgagctgcgccgccagcggattcaacatcaaggacacctacatccactgggtgaggcaggcccctggaaagggactggagtgggtggccagaatctaccccaccaacggctacacaagatacgccgacagcgtgaagggcagattcaccatcagcgccgacaccagcaagaacaccgcctacctgcagatgaacagcctgagagccgaggacacagccgtgtactactgctctagatggggaggcgagggcttctacgccatggactactggggacagggcacactggtgaccgtgtccagcgctagcaccaagggcccctccgtgttccccctggcccccagcagcaagagcaccagcggcggcacagccgctctgggctgcctggtcgaggactacttccccgagcccgtgaccgtgtcctggaacagcggagccctgacctccggcgtgcacaccttccccgccgtgctgcagagttctggcctgtatagcctgagcagcgtggtcaccgtgccttctagcagcctgggcacccagacctacatctgcaacgtgaaccacaagcccagcaacaccaaggtggacgagaaggtggagcccaagagctgcgacaaaactcacacatgcccaccgtgcccagcacctgaagctgcagggggaccgtcagtcttcctcttccccccaaaacccaaggacaccctcatgatctcccggacccctgaggtcacatgcgtggtggtggacgtgagccacgaagaccctgaggtcaagttcaactggtacgtggacggcgtggaggtgcataatgccaagacaaagccgcgggaggagcagtacaacagcacgtaccgtgtggtcagcgtcctcaccgtcctgcaccaggactggctgaatggcaaggagtacaagtgcaaggtctccaacaaagccctcggcgcccccatcgagaaaaccatctccaaagccaaagggcagccccgagaaccacaggtgtacaccctgcccccatgccgggatgagctgaccaagaaccaggtcagcctgtggtgcctggtcaaaggcttctatcccagcgacatcgccgtggagtgggagagcaatgggcagccggagaacaactacaagaccacgcctcccgtgctggactccgacggctccttcttcctctacagcaagctcaccgtggacaagagcaggtggcagcaggggaacgtcttctcatgctccgtgatgcatgaggctctgcacaaccactacacgcagaagagcctctccctgtctccgggtaaatga

SEQ ID NO: 166 - DNA, 1350 bp, Chimeric
caggtgcaattggttcaatctggtgctgaagtaaaaaaaccgggcgcttccgttaaagtgagctgcaaagcatccggatacaccttcacttcctattacatgcactgggttcgtcaagccccgggccagggtctggaatggatgggcatcattaacccaagcggtggctctacctcctacgcgcagaaattccagggtcgcgtcacgatgacccatgacactagcacctctaccgtttatatggagctgtccagcctgcgttctgaagatactgcagtgtactactgtgcacgctctttcttcactggtttccatctggactattggggtcaaggcaccctcgtaacggtttcttctgctagcaccaagggcccctccgtgttccccctggcccccagcagcaagagcaccagcggcggcacagccgctctgggctgcctggtcgaggactacttccccgagcccgtgaccgtgtcctggaacagcggagccctgacctccggcgtgcacaccttccccgccgtgctgcagagttctggcctgtatagcctgagcagcgtggtcaccgtgccttctagcagcctgggcacccagacctacatctgcaacgtgaaccacaagcccagcaacaccaaggtggacgagaaggtggagcccaagagctgcgacaaaactcacacatgcccaccgtgcccagcacctgaagctgcagggggaccgtcagtcttcctcttccccccaaaacccaaggacaccctcatgatctcccggacccctgaggtcacatgcgtggtggtggacgtgagccacgaagaccctgaggtcaagttcaactggtacgtggacggcgtggaggtgcataatgccaagacaaagccgcgggaggagcagtacaacagcacgtaccgtgtggtcagcgtcctcaccgtcctgcaccaggactggctgaatggcaaggagtacaagtgcaaggtctccaacaaagccctcggcgcccccatcgagaaaaccatctccaaagccaaagggcagccccgagaaccacaggtgtgcaccctgcccccatcccgggatgagctgaccaagaaccaggtcagcctctcgtgcgcagtcaaaggcttctatcccagcgacatcgccgtggagtgggagagcaatgggcagccggagaacaactacaagaccacgcctcccgtgctggactccgacggctccttcttcctcgtgagcaagctcaccgtggacaagagcaggtggcagcaggggaacgtcttctcatgctccgtgatgcatgaggctctgcacaaccactacacgcagaagagcctctccctgtctccgggtaaatga

SEQ ID NO: 167 - DNA, 651 bp, Chimeric
gaaatcgtgttaacgcagtctccaggcaccctgtctttgtctccaggggaaagagccaccctctcttgcagggccagtcagagtgttagcagcagctacttagcctggtaccagcagaaacctggccaggctcccaggctcctcatctatggagcatccagcagggccactggcatcccagacaggttcagtggcagtggatccgggacagacttcactctcaccatcagcagactggagcctgaagattttgcagtgtattactgtcagcagtataccaacgaacattattatacgttcggccaggggaccaaagtggaaatcaaacgtacggtggctgcaccatctgtcttcatcttcccgccatctgatcggaagttgaaatctggaactgcctctgttgtgtgcctgctgaataacttctatcccagagaggccaaagtacagtggaaggtggataacgccctccaatcgggtaactcccaggagagtgtcacagagcaggacagcaaggacagcacctacagcctcagcagcaccctgacgctgagcaaagcagactacgagaaacacaaagtctacgcctgcgaagtcacccatcagggcctgagctcgcccgtcacaaagagcttcaacaggggagagtgttag

SEQ ID NO: 168 - DNA, 2871 bp, Chimeric
caagtgcagctgaaagagtccggccctggactggtggcccctagccagagcctgagcatcacctgtaccgtgtccggcttcagcctgaccagctacggcgtgtcatgggtgcgccagcctccaggcaagtgtctggaatggctgggcatcatctggggcgacggcagcaccaattaccacagcgccctgatcagcagactgagcatctccaaggacaacagcaagagccaggtgttcctgaagctgaacagcctgcagaccgacgacaccgccacctactactgcgccaagggcatcaccaccgtggtggacgactactacgctatggactactggggccagggcaccagcgtgacagtgtctagcggaggcggaggatctggcggcggaggaagtggcggagggggatctgggggaggcggaagcgatatccagatgacccagagccctgccagcctgtctgcctctgtgggcgagacagtgaccatcacatgccgggccagcgagaacatcgacagctacctggcctggtatcagcagaagcagggcaagagcccccagctgctggtgtacgccgccacctttctggccgacgatgtgcccagcagattcagcggcagcggaagcggcacacagtacagcctgaagatcaactccctgcagagcgaggacgtggcccggtactactgccagcactactacagcaccccctacaccttcggctgcggcaccaagctggaaatcaaaggaggcggcggaagtgtgcacatgcccctgggcttcctgggccccagacaggccagagtcgtgaacggggggggcggaggcagtggggggggaggatcccaggccgtcgtgacccaggaacccagcctgacagtgtctcctggcggcaccgtgaccctgacatgtggcagttctacaggcgccgtgaccaccagcaactacgccaactgggtgcaggaaaagcccggccaggccttcagaggactgatcggcggcaccaacaagagagcccctggcacccctgccagattcagcggatctctgctgggaggaaaggccgccctgacactgtctggcgcccagccagaagatgaggccgagtactactgcgccctgtggtacagcaacctgtgggtgttcggcggaggcaccaagctgacagtgctgagcagcgcttccaccaagggacccagtgtgttccccctggcccccagctccaagtctacatccggtggcacagctgccctgggatgtctcgtgaaggactactttcctgagcctgtgacagtgtcttggaacagcggagccctgaccagcggagtgcacacattccctgcagtgctgcagagcagcggcctgtatagcctgagcagcgtcgtgaccgtgccttcctctagcctgggaacacagacatatatctgtaatgtgaatcataagcccagtaataccaaagtggataagaaagtggaacctaagagctgcgatggcggaggagggtccggaggcggagggtcccaggtgcaattggttcaatctggtgctgaagtaaaaaaaccgggcgcttccgttaaagtgagctgcaaagcatccggatacaccttcacttcctattacatgcactgggttcgtcaagccccgggccagggtctggaatggatgggcatcattaacccaagcggtggctctacctcctacgcgcagaaattccagggtcgcgtcacgatgacccatgacactagcacctctaccgtttatatggagctgtccagcctgcgttctgaagatactgcagtgtactactgtgcacgctctttcttcactggtttccatctggactattggggtcaaggcaccctcgtaacggtttcttctgctagcaccaagggcccctccgtgttccccctggcccccagcagcaagagcaccagcggcggcacagccgctctgggctgcctggtcgaggactacttccccgagcccgtgaccgtgtcctggaacagcggagccctgacctccggcgtgcacaccttccccgccgtgctgcagagttctggcctgtatagcctgagcagcgtggtcaccgtgccttctagcagcctgggcacccagacctacatctgcaacgtgaaccacaagcccagcaacaccaaggtggacgagaaggtggagcccaagagctgcgacaaaactcacacatgcccaccgtgcccagcacctgaagctgcagggggaccgtcagtcttcctcttccccccaaaacccaaggacaccctcatgatctcccggacccctgaggtcacatgcgtggtggtggacgtgagccacgaagaccctgaggtcaagttcaactggtacgtggacggcgtggaggtgcataatgccaagacaaagccgcgggaggagcagtacaacagcacgtaccgtgtggtcagcgtcctcaccgtcctgcaccaggactggctgaatggcaaggagtacaagtgcaaggtctccaacaaagccctcggcgcccccatcgagaaaaccatctccaaagccaaagggcagccccgagaaccacaggtgtacaccctgcccccatgccgggatgagctgaccaagaaccaggtcagcctgtggtgcctggtcaaaggcttctatcccagcgacatcgccgtggagtgggagagcaatgggcagccggagaacaactacaagaccacgcctcccgtgctggactccgacggctccttcttcctctacagcaagctcaccgtggacaagagcaggtggcagcaggggaacgtcttctcatgctccgtgatgcatgaggctctgcacaaccactacacgcagaagagcctctccctgtctccgggtaaatga

SEQ ID NO: 169 - DNA, 2857 bp, Chimeric
agagtccggccctggactggtggcccctagccagagcctgagcatcacctgtaccgtgtccggcttcagcctgaccagctacggcgtgtcatgggtgcgccagcctccaggcaagtgtctggaatggctgggcatcatctggggcgacggcagcaccaattaccacagcgccctgatcagcagactgagcatctccaaggacaacagcaagagccaggtgttcctgaagctgaacagcctgcagaccgacgacaccgccacctactactgcgccaagggcatcaccaccgtggtggacgactactacgctatggactactggggccagggcaccagcgtgacagtgtctagcggaggcggaggatctggcggcggaggaagtggcggagggggatctgggggaggcggaagcgatatccagatgacccagagccctgccagcctgtctgcctctgtgggcgagacagtgaccatcacatgccgggccagcgagaacatcgacagctacctggcctggtatcagcagaagcagggcaagagcccccagctgctggtgtacgccgccacctttctggccgacgatgtgcccagcagattcagcggcagcggaagcggcacacagtacagcctgaagatcaactccctgcagagcgaggacgtggcccggtactactgccagcactactacagcaccccctacaccttcggctgcggcaccaagctggaaatcaaaggcgggggaggctccggaggcggcggaagtggaggcggcggaagtggcggaggcggaggggggggaagtgggggcggaggcagtggggggggaggatcccaggccgtcgtgacccaggaacccagcctgacagtgtctcctggcggcaccgtgaccctgacatgtggcagttctacaggcgccgtgaccaccagcaactacgccaactgggtgcaggaaaagcccggccaggccttcagaggactgatcggcggcaccaacaagagagcccctggcacccctgccagattcagcggatctctgctgggaggaaaggccgccctgacactgtctggcgcccagccagaagatgaggccgagtactactgcgccctgtggtacagcaacctgtgggtgttcggcggaggcaccaagctgacagtgctgagcagcgcttccaccaagggacccagtgtgttccccctggcccccagctccaagtctacatccggtggcacagctgccctgggatgtctcgtgaaggactactttcctgagcctgtgacagtgtcttggaacagcggagccctgaccagcggagtgcacacattccctgcagtgctgcagagcagcggcctgtatagcctgagcagcgtcgtgaccgtgccttcctctagcctgggaacacagacatatatctgtaatgtgaatcataagcccagtaataccaaagtggataagaaagtggaacctaagagctgcgatggcggaggagggtctggaggcggagggtcccaggtgcaattggttcaatctggtgctgaagtaaaaaaaccgggcgcttccgttaaagtgagctgcaaagcatccggatacaccttcacttcctattacatgcactgggttcgtcaagccccgggccagggtctggaatggatgggcatcattaacccaagcggtggctctacctcctacgcgcagaaattccagggtcgcgtcacgatgacccatgacactagcacctctaccgtttatatggagctgtccagcctgcgttctgaagatactgcagtgtactactgtgcacgctctttcttcactggtttccatctggactattggggtcaaggcaccctcgtaacggtttcttctgctagcaccaagggcccctccgtgttccccctggcccccagcagcaagagcaccagcggcggcacagccgctctgggctgcctggtcgaggactacttccccgagcccgtgaccgtgtcctggaacagcggagccctgacctccggcgtgcacaccttccccgccgtgctgcagagttctggcctgtatagcctgagcagcgtggtcaccgtgccttctagcagcctgggcacccagacctacatctgcaacgtgaaccacaagcccagcaacaccaaggtggacgagaaggtggagcccaagagctgcgacaaaactcacacatgcccaccgtgcccagcacctgaagctgcagggggaccgtcagtcttcctcttccccccaaaacccaaggacaccctcatgatctcccggacccctgaggtcacatgcgtggtggtggacgtgagccacgaagaccctgaggtcaagttcaactggtacgtggacggcgtggaggtgcataatgccaagacaaagccgcgggaggagcagtacaacagcacgtaccgtgtggtcagcgtcctcaccgtcctgcaccaggactggctgaatggcaaggagtacaagtgcaaggtctccaacaaagccctcggcgcccccatcgagaaaaccatctccaaagccaaagggcagccccgagaaccacaggtgtacaccctgcccccatgccgggatgagctgaccaagaaccaggtcagcctgtggtgcctggtcaaaggcttctatcccagcgacatcgccgtggagtgggagagcaatgggcagccggagaacaactacaagaccacgcctcccgtgctggactccgacggctccttcttcctctacagcaagctcaccgtggacaagagcaggtggcagcaggggaacgtcttctcatgctccgtgatgcatgaggctctgcacaaccactacacgcagaagagcctctccctgtctccgggtaaatga

SEQ ID NO: 170 - DNA, 2025 bp, Chimeric
caggccgtcgtgacccaggaacccagcctgacagtgtctcctggcggcaccgtgaccctgacatgtggcagttctacaggcgccgtgaccaccagcaactacgccaactgggtgcaggaaaagcccggccaggccttcagaggactgatcggcggcaccaacaagagagcccctggcacccctgccagattcagcggatctctgctgggaggaaaggccgccctgacactgtctggcgcccagccagaagatgaggccgagtactactgcgccctgtggtacagcaacctgtgggtgttcggcggaggcaccaagctgacagtgctgagcagcgcttccaccaagggacccagtgtgttccccctggcccccagctccaagtctacatccggtggcacagctgccctgggatgtctcgtgaaggactactttcctgagcctgtgacagtgtcttggaacagcggagccctgaccagcggagtgcacacattccctgcagtgctgcagagcagcggcctgtatagcctgagcagcgtcgtgaccgtgccttcctctagcctgggaacacagacatatatctgtaatgtgaatcataagcccagtaataccaaagtggataagaaagtggaacctaagagctgcgatggcggaggagggtctggaggcggagggtcccaggtgcaattggttcaatctggtgctgaagtaaaaaaaccgggcgcttccgttaaagtgagctgcaaagcatccggatacaccttcacttcctattacatgcactgggttcgtcaagccccgggccagggtctggaatggatgggcatcattaacccaagcggtggctctacctcctacgcgcagaaattccagggtcgcgtcacgatgacccatgacactagcacctctaccgtttatatggagctgtccagcctgcgttctgaagatactgcagtgtactactgtgcacgctctttcttcactggtttccatctggactattggggtcaaggcaccctcgtaacggtttcttctgctagcaccaagggcccctccgtgttccccctggcccccagcagcaagagcaccagcggcggcacagccgctctgggctgcctggtcgaggactacttccccgagcccgtgaccgtgtcctggaacagcggagccctgacctccggcgtgcacaccttccccgccgtgctgcagagttctggcctgtatagcctgagcagcgtggtcaccgtgccttctagcagcctgggcacccagacctacatctgcaacgtgaaccacaagcccagcaacaccaaggtggacgagaaggtggagcccaagagctgcgacaaaactcacacatgcccaccgtgcccagcacctgaagctgcagggggaccgtcagtcttcctcttccccccaaaacccaaggacaccctcatgatctcccggacccctgaggtcacatgcgtggtggtggacgtgagccacgaagaccctgaggtcaagttcaactggtacgtggacggcgtggaggtgcataatgccaagacaaagccgcgggaggagcagtacaacagcacgtaccgtgtggtcagcgtcctcaccgtcctgcaccaggactggctgaatggcaaggagtacaagtgcaaggtctccaacaaagccctcggcgcccccatcgagaaaaccatctccaaagccaaagggcagccccgagaaccacaggtgtacaccctgcccccatgccgggatgagctgaccaagaaccaggtcagcctgtggtgcctggtcaaaggcttctatcccagcgacatcgccgtggagtgggagagcaatgggcagccggagaacaactacaagaccacgcctcccgtgctggactccgacggctccttcttcctctacagcaagctcaccgtggacaagagcaggtggcagcaggggaacgtcttctcatgctccgtgatgcatgaggctctgcacaaccactacacgcagaagagcctctccctgtctccgggtaaatga